European Patent Application EP 4 349 984 A1, published April 10, 2024. Title: PROBE AND USE THEREOF. Applicant: KYUSHU UNIVERSITY, NATIONAL UNIVERSITY CORPORATION. The sequence listing filed with the application follows.

SEQUENCE LISTING (751 sequences)

SEQ ID NO: 1 - DNA, 15 bp, Artificial sequence
  Synthetic nucleotides for probe
tgacgcgatacgcac

SEQ ID NO: 2 - DNA, 15 bp, Artificial sequence
  Synthetic nucleotides for probe
atgcgcagtatcgtg

SEQ ID NO: 3 - DNA, 15 bp, Artificial sequence
  Synthetic nucleotides for probe
tgcgctagtagtcgt

SEQ ID NO: 4 - DNA, 15 bp, Artificial sequence
  Synthetic nucleotides for probe
tcgagtcactatcgt

SEQ ID NO: 5 - DNA, 15 bp, Artificial sequence
  Synthetic nucleotides for probe
tgcgtctagctcata

SEQ ID NO: 6 - DNA, 15 bp, Artificial sequence
  Synthetic nucleotides for probe
acgtcgcatacgatc

SEQ ID NO: 7 - DNA, 15 bp, Artificial sequence
  Synthetic nucleotides for probe
tcgacactatacgat

SEQ ID NO: 8 - DNA, 15 bp, Artificial sequence
  Synthetic nucleotides for probe
tcgcgctatcgctag

SEQ ID NO: 9 - DNA, 15 bp, Artificial sequence
  Synthetic nucleotides for probe
tgtctactcgagcga

SEQ ID NO: 10 - DNA, 15 bp, Artificial sequence
  Synthetic nucleotides for probe
agtcgtcgagtcgca

SEQ ID NO: 11 - DNA, 15 bp, Artificial sequence
  Synthetic nucleotides for probe
actcgcatcgatata

SEQ ID NO: 12 - DNA, 15 bp, Artificial sequence
  Synthetic nucleotides for probe
tcgcgagtagagcac

SEQ ID NO: 13 - DNA, 15 bp, Artificial sequence
  Synthetic nucleotides for probe
agtatactcgcgatg

SEQ ID NO: 14 - DNA, 15 bp, Artificial sequence
  Synthetic nucleotides for probe
tacgagtgcacgacg

SEQ ID NO: 15 - DNA, 15 bp, Artificial sequence
  Synthetic nucleotides for probe
tagtatgcgcgtcta

SEQ ID NO: 16 - DNA, 15 bp, Artificial sequence
  Synthetic nucleotides for probe
acgtgagtcgtagtg

SEQ ID NO: 17 - DNA, 15 bp, Artificial sequence
  Synthetic nucleotides for probe
acgtactcgtactac

SEQ ID NO: 18 - DNA, 15 bp, Artificial sequence
  Synthetic nucleotides for probe
acgcacgactcatgc

SEQ ID NO: 19 - DNA, 15 bp, Artificial sequence
  Synthetic nucleotides for probe
atcgagtagagatcg

SEQ ID NO: 20 - DNA, 15 bp, Artificial sequence
  Synthetic nucleotides for probe
tgatcgtacgcgcag

SEQ ID NO: 21 - DNA, 15 bp, Artificial sequence
  Synthetic nucleotides for probe
tatgtcagacgacgc

SEQ ID NO: 22 - DNA, 15 bp, Artificial sequence
  Synthetic nucleotides for probe
tatcgctcgtcgatc

SEQ ID NO: 23 - DNA, 15 bp, Artificial sequence
  Synthetic nucleotides for probe
tgctctagcgatacg

SEQ ID NO: 24 - DNA, 15 bp, Artificial sequence
  Synthetic nucleotides for probe
tacgtcacgcgtctg

SEQ ID NO: 25 - DNA, 15 bp, Artificial sequence
  Synthetic nucleotides for probe
tcgtatgtatcgtga

SEQ ID NO: 26 - DNA, 15 bp, Artificial sequence
  Synthetic nucleotides for probe
atcgagagatcgacg

SEQ ID NO: 27 - DNA, 15 bp, Artificial sequence
  Synthetic nucleotides for probe
tactagtcgtgagat

SEQ ID NO: 28 - DNA, 15 bp, Artificial sequence
  Synthetic nucleotides for probe
ttcgaatcttacgtc

SEQ ID NO: 29 - DNA, 15 bp, Artificial sequence
  Synthetic nucleotides for probe
aattagctccggata

SEQ ID NO: 30 - DNA, 15 bp, Artificial sequence
  Synthetic nucleotides for probe
atgatcggtgtacgt

SEQ ID NO: 31 - DNA, 15 bp, Artificial sequence
  Synthetic nucleotides for probe
taccttagtacgcgg

SEQ ID NO: 32 - DNA, 15 bp, Artificial sequence
  Synthetic nucleotides for probe
taatggttcaacgac

SEQ ID NO: 33 - DNA, 15 bp, Artificial sequence
  Synthetic nucleotides for probe
ttctacgcgttcgat

SEQ ID NO: 34 - DNA, 15 bp, Artificial sequence
  Synthetic nucleotides for probe
aatactcgttgaccg

SEQ ID NO: 35 - DNA, 15 bp, Artificial sequence
  Synthetic nucleotides for probe
tacggcgatgcttgc

SEQ ID NO: 36 - DNA, 15 bp, Artificial sequence
  Synthetic nucleotides for probe
acgctacgtgttagc

SEQ ID NO: 37 - DNA, 15 bp, Artificial sequence
  Synthetic nucleotides for probe
tcgtattatcctcga

SEQ ID NO: 38 - DNA, 15 bp, Artificial sequence
  Synthetic nucleotides for probe
tatgacaacgcgtat

SEQ ID NO: 39 - DNA, 15 bp, Artificial sequence
  Synthetic nucleotides for probe
atagagcgaacgacg

SEQ ID NO: 40 - DNA, 15 bp, Artificial sequence
  Synthetic nucleotides for probe
aatcgtggccagtcg

SEQ ID NO: 41 - DNA, 15 bp, Artificial sequence
  Synthetic nucleotides for probe
attacacgccgactc

SEQ ID NO: 42 - DNA, 15 bp, Artificial sequence
  Synthetic nucleotides for probe
aggtaccggatacgc

SEQ ID NO: 43 - DNA, 15 bp, Artificial sequence
  Synthetic nucleotides for probe
tgcacgtaattcgac

SEQ ID NO: 44 - DNA, 15 bp, Artificial sequence
  Synthetic nucleotides for probe
agaatccggtagcgc

SEQ ID NO: 45 - DNA, 15 bp, Artificial sequence
  Synthetic nucleotides for probe
attgtacgcctatcg

SEQ ID NO: 46 - DNA, 15 bp, Artificial sequence
  Synthetic nucleotides for probe
tgtgcgtacattacg

SEQ ID NO: 47 - DNA, 15 bp, Artificial sequence
  Synthetic nucleotides for probe
tcgtgtcaagtacgt

SEQ ID NO: 48 - DNA, 15 bp, Artificial sequence
  Synthetic nucleotides for probe
agctaacgcgccgaa

SEQ ID NO: 49 - DNA, 15 bp, Artificial sequence
  Synthetic nucleotides for probe
tacgctaattcgtcg

SEQ ID NO: 50 - DNA, 15 bp, Artificial sequence
  Synthetic nucleotides for probe
ttgcgcgtacataca

SEQ ID NO: 51 - DNA, 15 bp, Artificial sequence
  Synthetic nucleotides for probe
tgaacgagagtcgat

SEQ ID NO: 52 - DNA, 15 bp, Artificial sequence
  Synthetic nucleotides for probe
taccgtagcacgaca

SEQ ID NO: 53 - DNA, 15 bp, Artificial sequence
  Synthetic nucleotides for probe
atatctctggcgtac

SEQ ID NO: 54 - DNA, 15 bp, Artificial sequence
  Synthetic nucleotides for probe
agtaaccgcgtatgg

SEQ ID NO: 55 - DNA, 15 bp, Artificial sequence
  Synthetic nucleotides for probe
atagttaagaccgac

SEQ ID NO: 56 - DNA, 15 bp, Artificial sequence
  Synthetic nucleotides for probe
aggtcgacagtatac

SEQ ID NO: 57 - DNA, 15 bp, Artificial sequence
  Synthetic nucleotides for probe
taaccgtctcgtatc

SEQ ID NO: 58 - DNA, 15 bp, Artificial sequence
  Synthetic nucleotides for probe
tgcgtatgcgattag

SEQ ID NO: 59 - DNA, 15 bp, Artificial sequence
  Synthetic nucleotides for probe
ttacgttaatccgac

SEQ ID NO: 60 - DNA, 15 bp, Artificial sequence
  Synthetic nucleotides for probe
accgcgtggtaattc

SEQ ID NO: 61 - DNA, 15 bp, Artificial sequence
  Synthetic nucleotides for probe
tcgtaactatacgtc

SEQ ID NO: 62 - DNA, 15 bp, Artificial sequence
  Synthetic nucleotides for probe
acgcatacggtagac

SEQ ID NO: 63 - DNA, 15 bp, Artificial sequence
  Synthetic nucleotides for probe
actaaccgaccgtac

SEQ ID NO: 64 - DNA, 15 bp, Artificial sequence
  Synthetic nucleotides for probe
taccggtaacgacgt

SEQ ID NO: 65 - DNA, 15 bp, Artificial sequence
  Synthetic nucleotides for probe
ttcggccgcgtatat

SEQ ID NO: 66 - DNA, 15 bp, Artificial sequence
  Synthetic nucleotides for probe
atacgctcgcgaaca

SEQ ID NO: 67 - DNA, 15 bp, Artificial sequence
  Synthetic nucleotides for probe
tagtaacgttgcgtg

SEQ ID NO: 68 - DNA, 15 bp, Artificial sequence
  Synthetic nucleotides for probe
ttcggacgtacctaa

SEQ ID NO: 69 - DNA, 15 bp, Artificial sequence
  Synthetic nucleotides for probe
agttatcctggcgcg

SEQ ID NO: 70 - DNA, 15 bp, Artificial sequence
  Synthetic nucleotides for probe
tcgtaagtcggtgtc

SEQ ID NO: 71 - DNA, 15 bp, Artificial sequence
  Synthetic nucleotides for probe
accttaacgcggata

SEQ ID NO: 72 - DNA, 15 bp, Artificial sequence
  Synthetic nucleotides for probe
aatactatcgcgcag

SEQ ID NO: 73 - DNA, 15 bp, Artificial sequence
  Synthetic nucleotides for probe
agacttaccgcgatc

SEQ ID NO: 74 - DNA, 15 bp, Artificial sequence
  Synthetic nucleotides for probe
atgccataattcgcg

SEQ ID NO: 75 - DNA, 15 bp, Artificial sequence
  Synthetic nucleotides for probe
acggcgaacgtatga

SEQ ID NO: 76 - DNA, 15 bp, Artificial sequence
  Synthetic nucleotides for probe
agtgcggtgaccgta

SEQ ID NO: 77 - DNA, 15 bp, Artificial sequence
  Synthetic nucleotides for probe
ttacgatatagcgcc

SEQ ID NO: 78 - DNA, 15 bp, Artificial sequence
  Synthetic nucleotides for probe
ttcggattcataacc

SEQ ID NO: 79 - DNA, 15 bp, Artificial sequence
  Synthetic nucleotides for probe
taacggagttcggct

SEQ ID NO: 80 - DNA, 15 bp, Artificial sequence
  Synthetic nucleotides for probe
ttatgcaagcgtacc

SEQ ID NO: 81 - DNA, 15 bp, Artificial sequence
  Synthetic nucleotides for probe
acaaccggtcgacct

SEQ ID NO: 82 - DNA, 15 bp, Artificial sequence
  Synthetic nucleotides for probe
ttgtatcggcgacca

SEQ ID NO: 83 - DNA, 15 bp, Artificial sequence
  Synthetic nucleotides for probe
tcgataggtgcacgg

SEQ ID NO: 84 - DNA, 15 bp, Artificial sequence
  Synthetic nucleotides for probe
acgacacctcgtatt

SEQ ID NO: 85 - DNA, 15 bp, Artificial sequence
  Synthetic nucleotides for probe
aaggcgatatacgat

SEQ ID NO: 86 - DNA, 15 bp, Artificial sequence
  Synthetic nucleotides for probe
tagtcgcttacgcgt

SEQ ID NO: 87 - DNA, 15 bp, Artificial sequence
  Synthetic nucleotides for probe
taccgcgatagccta

SEQ ID NO: 88 - DNA, 15 bp, Artificial sequence
  Synthetic nucleotides for probe
atgcgattcgcgatt

SEQ ID NO: 89 - DNA, 15 bp, Artificial sequence
  Synthetic nucleotides for probe
attgattccgacgta

SEQ ID NO: 90 - DNA, 15 bp, Artificial sequence
  Synthetic nucleotides for probe
ataattgcgaagacg

SEQ ID NO: 91 - DNA, 15 bp, Artificial sequence
  Synthetic nucleotides for probe
aatggtacacgatcg

SEQ ID NO: 92 - DNA, 15 bp, Artificial sequence
  Synthetic nucleotides for probe
tctccgccgattacg

SEQ ID NO: 93 - DNA, 15 bp, Artificial sequence
  Synthetic nucleotides for probe
tcggttctattatcg

SEQ ID NO: 94 - DNA, 15 bp, Artificial sequence
  Synthetic nucleotides for probe
tcgtagtccaactta

SEQ ID NO: 95 - DNA, 15 bp, Artificial sequence
  Synthetic nucleotides for probe
aggcggttacgaatt

SEQ ID NO: 96 - DNA, 15 bp, Artificial sequence
  Synthetic nucleotides for probe
tagtaatctcgttcg

SEQ ID NO: 97 - DNA, 15 bp, Artificial sequence
  Synthetic nucleotides for probe
aaccactatatacgc

SEQ ID NO: 98 - DNA, 15 bp, Artificial sequence
  Synthetic nucleotides for probe
taacaggcctagcga

SEQ ID NO: 99 - DNA, 15 bp, Artificial sequence
  Synthetic nucleotides for probe
accgagcgactgtaa

SEQ ID NO: 100 - DNA, 15 bp, Artificial sequence
  Synthetic nucleotides for probe
tagtgtatccgtccg

SEQ ID NO: 101 - DNA, 15 bp, Artificial sequence
  Synthetic nucleotides for probe
aggtgtcggcaatcg

SEQ ID NO: 102 - DNA, 15 bp, Artificial sequence
  Synthetic nucleotides for probe
tcgcgtattcatatc

SEQ ID NO: 103 - DNA, 15 bp, Artificial sequence
  Synthetic nucleotides for probe
tctaccagccgctaa

SEQ ID NO: 104 - DNA, 15 bp, Artificial sequence
  Synthetic nucleotides for probe
actccgcatgttccg

SEQ ID NO: 105 - DNA, 15 bp, Artificial sequence
  Synthetic nucleotides for probe
actgatgtaacggcg

SEQ ID NO: 106 - DNA, 15 bp, Artificial sequence
  Synthetic nucleotides for probe
tccgatatcactcgg

SEQ ID NO: 107 - DNA, 15 bp, Artificial sequence
  Synthetic nucleotides for probe
taatctacgtcaggc

SEQ ID NO: 108 - DNA, 15 bp, Artificial sequence
  Synthetic nucleotides for probe
tagtcttagttcgca

SEQ ID NO: 109 - DNA, 15 bp, Artificial sequence
  Synthetic nucleotides for probe
tagcgttcgtcgcaa

SEQ ID NO: 110 - DNA, 15 bp, Artificial sequence
  Synthetic nucleotides for probe
tcgctctgtcgcaat

SEQ ID NO: 111 - DNA, 15 bp, Artificial sequence
  Synthetic nucleotides for probe
ttaacgtgatgtcgg

SEQ ID NO: 112 - DNA, 15 bp, Artificial sequence
  Synthetic nucleotides for probe
acaccgtagcgtcat

SEQ ID NO: 113 - DNA, 15 bp, Artificial sequence
  Synthetic nucleotides for probe
tcgtattaagcgcgt

SEQ ID NO: 114 - DNA, 15 bp, Artificial sequence
  Synthetic nucleotides for probe
taaccttgtacgcga

SEQ ID NO: 115 - DNA, 15 bp, Artificial sequence
  Synthetic nucleotides for probe
accgtgatcgattgg

SEQ ID NO: 116 - DNA, 15 bp, Artificial sequence
  Synthetic nucleotides for probe
ttcgcaagttagccg

SEQ ID NO: 117 - DNA, 15 bp, Artificial sequence
  Synthetic nucleotides for probe
attacgcgatgcgga

SEQ ID NO: 118 - DNA, 15 bp, Artificial sequence
  Synthetic nucleotides for probe
tcgcgctagattaga

SEQ ID NO: 119 - DNA, 15 bp, Artificial sequence
  Synthetic nucleotides for probe
ttgcggttactcgcg

SEQ ID NO: 120 - DNA, 15 bp, Artificial sequence
  Synthetic nucleotides for probe
ataccgctatccgaa

SEQ ID NO: 121 - DNA, 15 bp, Artificial sequence
  Synthetic nucleotides for probe
acgtaacaacgtaag

SEQ ID NO: 122 - DNA, 15 bp, Artificial sequence
  Synthetic nucleotides for probe
ttcgactggttgcgt

SEQ ID NO: 123 - DNA, 15 bp, Artificial sequence
  Synthetic nucleotides for probe
tacggtactactcgt

SEQ ID NO: 124 - DNA, 15 bp, Artificial sequence
  Synthetic nucleotides for probe
tacaactgctcgata

SEQ ID NO: 125 - DNA, 15 bp, Artificial sequence
  Synthetic nucleotides for probe
ttaatacgcgacgtt

SEQ ID NO: 126 - DNA, 15 bp, Artificial sequence
  Synthetic nucleotides for probe
tcggagtatcggact

SEQ ID NO: 127 - DNA, 15 bp, Artificial sequence
  Synthetic nucleotides for probe
ttccgttcgattgct

SEQ ID NO: 128 - DNA, 15 bp, Artificial sequence
  Synthetic nucleotides for probe
tagtacgcgtctgcc

SEQ ID NO: 129 - DNA, 15 bp, Artificial sequence
  Synthetic nucleotides for probe
tctatacgcgtcggt

SEQ ID NO: 130 - DNA, 15 bp, Artificial sequence
  Synthetic nucleotides for probe
tccgacgtatactat

SEQ ID NO: 131 - DNA, 15 bp, Artificial sequence
  Synthetic nucleotides for probe
agcgatagtaattcg

SEQ ID NO: 132 - DNA, 15 bp, Artificial sequence
  Synthetic nucleotides for probe
atcggtattccacaa

SEQ ID NO: 133 - DNA, 15 bp, Artificial sequence
  Synthetic nucleotides for probe
taaggtaaccagacg

SEQ ID NO: 134 - DNA, 15 bp, Artificial sequence
  Synthetic nucleotides for probe
tccgtaatacgcaat

SEQ ID NO: 135 - DNA, 15 bp, Artificial sequence
  Synthetic nucleotides for probe
aattcgtccggatta

SEQ ID NO: 136 - DNA, 15 bp, Artificial sequence
  Synthetic nucleotides for probe
tacgtcgctagtaat

SEQ ID NO: 137 - DNA, 15 bp, Artificial sequence
  Synthetic nucleotides for probe
tcgttggcgagaata

SEQ ID NO: 138 - DNA, 15 bp, Artificial sequence
  Synthetic nucleotides for probe
acgaactcttatcgt

SEQ ID NO: 139 - DNA, 15 bp, Artificial sequence
  Synthetic nucleotides for probe
tacggtaacattacg

SEQ ID NO: 140 - DNA, 15 bp, Artificial sequence
  Synthetic nucleotides for probe
tctacgcggattgcc

SEQ ID NO: 141 - DNA, 15 bp, Artificial sequence
  Synthetic nucleotides for probe
aggcggttcgctagt

SEQ ID NO: 142 - DNA, 15 bp, Artificial sequence
  Synthetic nucleotides for probe
atgattagcgttcgg

SEQ ID NO: 143 - DNA, 15 bp, Artificial sequence
  Synthetic nucleotides for probe
aacgacatacgtcgt

SEQ ID NO: 144 - DNA, 15 bp, Artificial sequence
  Synthetic nucleotides for probe
taactgcgtacgata

SEQ ID NO: 145 - DNA, 15 bp, Artificial sequence
  Synthetic nucleotides for probe
taagataatcgccga

SEQ ID NO: 146 - DNA, 15 bp, Artificial sequence
  Synthetic nucleotides for probe
aattcgcgaccgtgc

SEQ ID NO: 147 - DNA, 15 bp, Artificial sequence
  Synthetic nucleotides for probe
aagcgatacgctacc

SEQ ID NO: 148 - DNA, 15 bp, Artificial sequence
  Synthetic nucleotides for probe
aacgatacacgaggt

SEQ ID NO: 149 - DNA, 15 bp, Artificial sequence
  Synthetic nucleotides for probe
atccgattacgaggt

SEQ ID NO: 150 - DNA, 15 bp, Artificial sequence
  Synthetic nucleotides for probe
ttcgccggtcaattg

SEQ ID NO: 151 - DNA, 15 bp, Artificial sequence
  Synthetic nucleotides for probe
tagccgactatcgac

SEQ ID NO: 152 - DNA, 15 bp, Artificial sequence
  Synthetic nucleotides for probe
ttgcactatacggcg

SEQ ID NO: 153 - DNA, 15 bp, Artificial sequence
  Synthetic nucleotides for probe
agtcgataagagccg

SEQ ID NO: 154 - DNA, 15 bp, Artificial sequence
  Synthetic nucleotides for probe
agttaaggcgtacga

SEQ ID NO: 155 - DNA, 15 bp, Artificial sequence
  Synthetic nucleotides for probe
acgtcaacggatgat

SEQ ID NO: 156 - DNA, 15 bp, Artificial sequence
  Synthetic nucleotides for probe
ataagtcgtaacacg

SEQ ID NO: 157 - DNA, 15 bp, Artificial sequence
  Synthetic nucleotides for probe
tattcggaccgtcgt

SEQ ID NO: 158 - DNA, 15 bp, Artificial sequence
  Synthetic nucleotides for probe
ttagcttccatacgg

SEQ ID NO: 159 - DNA, 15 bp, Artificial sequence
  Synthetic nucleotides for probe
aataaccgtaccgga

SEQ ID NO: 160 - DNA, 15 bp, Artificial sequence
  Synthetic nucleotides for probe
agctcgattagacgc

SEQ ID NO: 161 - DNA, 15 bp, Artificial sequence
  Synthetic nucleotides for probe
tattaggcgcagtcg

SEQ ID NO: 162 - DNA, 15 bp, Artificial sequence
  Synthetic nucleotides for probe
tcatgcgccgtactg

SEQ ID NO: 163 - DNA, 15 bp, Artificial sequence
  Synthetic nucleotides for probe
atgtgatactcgcgg

SEQ ID NO: 164 - DNA, 15 bp, Artificial sequence
  Synthetic nucleotides for probe
tcgtaacgattgtcg

SEQ ID NO: 165 - DNA, 15 bp, Artificial sequence
  Synthetic nucleotides for probe
attggcgaataggcg

SEQ ID NO: 166 - DNA, 15 bp, Artificial sequence
  Synthetic nucleotides for probe
acatcgtagaccgaa

SEQ ID NO: 167 - DNA, 15 bp, Artificial sequence
  Synthetic nucleotides for probe
acgtatcgagaagcg

SEQ ID NO: 168 - DNA, 15 bp, Artificial sequence
  Synthetic nucleotides for probe
attacgcgcttgtaa

SEQ ID NO: 169 - DNA, 15 bp, Artificial sequence
  Synthetic nucleotides for probe
ttatacgactctcgc

SEQ ID NO: 170 - DNA, 15 bp, Artificial sequence
  Synthetic nucleotides for probe
ttcgctagttcgtct

SEQ ID NO: 171 - DNA, 15 bp, Artificial sequence
  Synthetic nucleotides for probe
agtcgcgcatagatt

SEQ ID NO: 172 - DNA, 15 bp, Artificial sequence
  Synthetic nucleotides for probe
tcatataagcgtagg

SEQ ID NO: 173 - DNA, 15 bp, Artificial sequence
  Synthetic nucleotides for probe
tactgcgagttatcg

SEQ ID NO: 174 - DNA, 15 bp, Artificial sequence
  Synthetic nucleotides for probe
taattccactcgacg

SEQ ID NO: 175 - DNA, 15 bp, Artificial sequence
  Synthetic nucleotides for probe
ttacgcaacgcgagt

SEQ ID NO: 176 - DNA, 15 bp, Artificial sequence
  Synthetic nucleotides for probe
ttaatcggttaccgc

SEQ ID NO: 177 - DNA, 15 bp, Artificial sequence
  Synthetic nucleotides for probe
ttatcctatgagcgc

SEQ ID NO: 178 - DNA, 15 bp, Artificial sequence
  Synthetic nucleotides for probe
attaagcttcgctcg

SEQ ID NO: 179 - DNA, 15 bp, Artificial sequence
  Synthetic nucleotides for probe
acttaccactagcga

SEQ ID NO: 180 - DNA, 15 bp, Artificial sequence
  Synthetic nucleotides for probe
tagaattacgcggaa

SEQ ID NO: 181 - DNA, 15 bp, Artificial sequence
  Synthetic nucleotides for probe
tgccggttaggtaat

SEQ ID NO: 182 - DNA, 15 bp, Artificial sequence
  Synthetic nucleotides for probe
tgcatcggtcttcgt

SEQ ID NO: 183 - DNA, 15 bp, Artificial sequence
  Synthetic nucleotides for probe
tgcacaatatccgcg

SEQ ID NO: 184 - DNA, 15 bp, Artificial sequence
  Synthetic nucleotides for probe
aagattaacgcacgg

SEQ ID NO: 185 - DNA, 15 bp, Artificial sequence
  Synthetic nucleotides for probe
acgcgtaccattgac

SEQ ID NO: 186 - DNA, 15 bp, Artificial sequence
  Synthetic nucleotides for probe
tggtctcaatagtcg

SEQ ID NO: 187 - DNA, 15 bp, Artificial sequence
  Synthetic nucleotides for probe
tcatcgatccgactt

SEQ ID NO: 188 - DNA, 15 bp, Artificial sequence
  Synthetic nucleotides for probe
acaacgtcgataggt

SEQ ID NO: 189 - DNA, 15 bp, Artificial sequence
  Synthetic nucleotides for probe
atcttatgacgagcg

SEQ ID NO: 190 - DNA, 15 bp, Artificial sequence
  Synthetic nucleotides for probe
agctagtaacggcga

SEQ ID NO: 191 - DNA, 15 bp, Artificial sequence
  Synthetic nucleotides for probe
atgtgtaatcgaacg

SEQ ID NO: 192 - DNA, 15 bp, Artificial sequence
  Synthetic nucleotides for probe
atgcataaggtggcg

SEQ ID NO: 193 - DNA, 15 bp, Artificial sequence
  Synthetic nucleotides for probe
acgcgatcaacctat

SEQ ID NO: 194 - DNA, 15 bp, Artificial sequence
  Synthetic nucleotides for probe
tgcgaatatatggcg

SEQ ID NO: 195 - DNA, 15 bp, Artificial sequence
  Synthetic nucleotides for probe
tatacgccagataga

SEQ ID NO: 196 - DNA, 15 bp, Artificial sequence
  Synthetic nucleotides for probe
acgtctactatcgga

SEQ ID NO: 197 - DNA, 15 bp, Artificial sequence
  Synthetic nucleotides for probe
aatcacgaggcgact

SEQ ID NO: 198 - DNA, 15 bp, Artificial sequence
  Synthetic nucleotides for probe
acgcgatgatcgtaa

SEQ ID NO: 199 - DNA, 15 bp, Artificial sequence
  Synthetic nucleotides for probe
tcgtgactatacgtt

SEQ ID NO: 200 - DNA, 15 bp, Artificial sequence
  Synthetic nucleotides for probe
atccgaacttagcgg

SEQ ID NO: 201 - DNA, 15 bp, Artificial sequence
  Synthetic nucleotides for probe
taggtcgacaccgat

SEQ ID NO: 202 - DNA, 15 bp, Artificial sequence
  Synthetic nucleotides for probe
ataggcgtagtacta

SEQ ID NO: 203 - DNA, 15 bp, Artificial sequence
  Synthetic nucleotides for probe
acgtcgcggctatgt

SEQ ID NO: 204 - DNA, 15 bp, Artificial sequence
  Synthetic nucleotides for probe
tagtagcgttacgcg

SEQ ID NO: 205 - DNA, 15 bp, Artificial sequence
  Synthetic nucleotides for probe
tgttaacgtagagcg

SEQ ID NO: 206 - DNA, 15 bp, Artificial sequence
  Synthetic nucleotides for probe
tctatgcgtcgcctt

SEQ ID NO: 207 - DNA, 15 bp, Artificial sequence
  Synthetic nucleotides for probe
accgttatgcacggt

SEQ ID NO: 208 - DNA, 15 bp, Artificial sequence
  Synthetic nucleotides for probe
tagtaccagccgtag

SEQ ID NO: 209 - DNA, 15 bp, Artificial sequence
  Synthetic nucleotides for probe
tcgtcggatatcgac

SEQ ID NO: 210 - DNA, 15 bp, Artificial sequence
  Synthetic nucleotides for probe
ttgcgcgttggaacg

SEQ ID NO: 211 - DNA, 15 bp, Artificial sequence
  Synthetic nucleotides for probe
ttagacgcacctacg

SEQ ID NO: 212 - DNA, 15 bp, Artificial sequence
  Synthetic nucleotides for probe
tattaggtcgtagcg

SEQ ID NO: 213 - DNA, 15 bp, Artificial sequence
  Synthetic nucleotides for probe
actccgaacgtatag

SEQ ID NO: 214 - DNA, 15 bp, Artificial sequence
  Synthetic nucleotides for probe
aacgattagcgacgt

SEQ ID NO: 215 - DNA, 15 bp, Artificial sequence
  Synthetic nucleotides for probe
atataccggaagatc

SEQ ID NO: 216 - DNA, 15 bp, Artificial sequence
  Synthetic nucleotides for probe
tgaatccgtgctagt

SEQ ID NO: 217 - DNA, 15 bp, Artificial sequence
  Synthetic nucleotides for probe
attagcggaattacc

SEQ ID NO: 218 - DNA, 15 bp, Artificial sequence
  Synthetic nucleotides for probe
actatcctcgtgacg

SEQ ID NO: 219 - DNA, 15 bp, Artificial sequence
  Synthetic nucleotides for probe
tgttatcgtgacgcc

SEQ ID NO: 220 - DNA, 15 bp, Artificial sequence
  Synthetic nucleotides for probe
tacttacgaatccgg

SEQ ID NO: 221 - DNA, 15 bp, Artificial sequence
  Synthetic nucleotides for probe
aagaagcgcgtactc

SEQ ID NO: 222 - DNA, 15 bp, Artificial sequence
  Synthetic nucleotides for probe
acgtgtcggtattgg

SEQ ID NO: 223 - DNA, 15 bp, Artificial sequence
  Synthetic nucleotides for probe
taacgcttcaatcgc

SEQ ID NO: 224 - DNA, 15 bp, Artificial sequence
  Synthetic nucleotides for probe
tcaatcgtcacggtc

SEQ ID NO: 225 - DNA, 15 bp, Artificial sequence
  Synthetic nucleotides for probe
acggaccggataggt

SEQ ID NO: 226 - DNA, 15 bp, Artificial sequence
  Synthetic nucleotides for probe
agtcgacaatcggct

SEQ ID NO: 227 - DNA, 15 bp, Artificial sequence
  Synthetic nucleotides for probe
tctaattatgcggcc

SEQ ID NO: 228 - DNA, 15 bp, Artificial sequence
  Synthetic nucleotides for probe
tgtagctatacggtc

SEQ ID NO: 229 - DNA, 15 bp, Artificial sequence
  Synthetic nucleotides for probe
aacgtaatacagcgg

SEQ ID NO: 230 - DNA, 15 bp, Artificial sequence
  Synthetic nucleotides for probe
taattaggcgtcgag

SEQ ID NO: 231 - DNA, 15 bp, Artificial sequence
  Synthetic nucleotides for probe
ttcgaacactattcg

SEQ ID NO: 232 - DNA, 15 bp, Artificial sequence
  Synthetic nucleotides for probe
tgttatacgaaggcg

SEQ ID NO: 233 - DNA, 15 bp, Artificial sequence
  Synthetic nucleotides for probe
tcgtctgttgcgtcg

SEQ ID NO: 234 - DNA, 15 bp, Artificial sequence
  Synthetic nucleotides for probe
acgcgcctatcttac

SEQ ID NO: 235 - DNA, 15 bp, Artificial sequence
  Synthetic nucleotides for probe
aagttccgatgctcg

SEQ ID NO: 236 - DNA, 15 bp, Artificial sequence
  Synthetic nucleotides for probe
agtgttgatcgtcgc

SEQ ID NO: 237 - DNA, 15 bp, Artificial sequence
  Synthetic nucleotides for probe
ttatcgccgtatgcg

SEQ ID NO: 238 - DNA, 15 bp, Artificial sequence
  Synthetic nucleotides for probe
atacgcgattacgaa

SEQ ID NO: 239 - DNA, 15 bp, Artificial sequence
  Synthetic nucleotides for probe
tagtacatagcggtc

SEQ ID NO: 240 - DNA, 15 bp, Artificial sequence
  Synthetic nucleotides for probe
taggttgattacgcg

SEQ ID NO: 241 - DNA, 15 bp, Artificial sequence
  Synthetic nucleotides for probe
acggttacgtcggca

SEQ ID NO: 242 - DNA, 15 bp, Artificial sequence
  Synthetic nucleotides for probe
aactacgcgagccat

SEQ ID NO: 243 - DNA, 15 bp, Artificial sequence
  Synthetic nucleotides for probe
acgtgtcgttcaacg

SEQ ID NO: 244 - DNA, 15 bp, Artificial sequence
  Synthetic nucleotides for probe
tgatgccggtatcgg

SEQ ID NO: 245 - DNA, 15 bp, Artificial sequence
  Synthetic nucleotides for probe
acatgtcgcgtaatc

SEQ ID NO: 246 - DNA, 15 bp, Artificial sequence
  Synthetic nucleotides for probe
aacgatatctcgctc

SEQ ID NO: 247 - DNA, 15 bp, Artificial sequence
  Synthetic nucleotides for probe
ataagccggcgaaca

SEQ ID NO: 248 - DNA, 15 bp, Artificial sequence
  Synthetic nucleotides for probe
agcgcgtaggattga

SEQ ID NO: 249 - DNA, 15 bp, Artificial sequence
  Synthetic nucleotides for probe
tcgcgtctggcaata

SEQ ID NO: 250 - DNA, 15 bp, Artificial sequence
  Synthetic nucleotides for probe
tggccggaacgatag

SEQ ID NO: 251 - DNA, 15 bp, Artificial sequence
  Synthetic nucleotides for probe
aatatacggtacgtc

SEQ ID NO: 252 - DNA, 15 bp, Artificial sequence
  Synthetic nucleotides for probe
ttaacggcgcgatgg

SEQ ID NO: 253 - DNA, 15 bp, Artificial sequence
  Synthetic nucleotides for probe
accgtaaggtcgcag

SEQ ID NO: 254 - DNA, 15 bp, Artificial sequence
  Synthetic nucleotides for probe
aggtcgacggctatt

SEQ ID NO: 255 - DNA, 15 bp, Artificial sequence
  Synthetic nucleotides for probe
agttactcacgccgg

SEQ ID NO: 256 - DNA, 15 bp, Artificial sequence
  Synthetic nucleotides for probe
acggcgcatcgttag

SEQ ID NO: 257 - DNA, 15 bp, Artificial sequence
  Synthetic nucleotides for probe
aggttacggtctcga

SEQ ID NO: 258 - DNA, 15 bp, Artificial sequence
  Synthetic nucleotides for probe
tattcggtcacctat

SEQ ID NO: 259 - DNA, 15 bp, Artificial sequence
  Synthetic nucleotides for probe
ttaggttcgtcgttg

SEQ ID NO: 260 - DNA, 15 bp, Artificial sequence
  Synthetic nucleotides for probe
acgcaggaatactcg

SEQ ID NO: 261 - DNA, 15 bp, Artificial sequence
  Synthetic nucleotides for probe
agcgattacatgcgc

SEQ ID NO: 262 - DNA, 15 bp, Artificial sequence
  Synthetic nucleotides for probe
agcgcgaccatacgt

SEQ ID NO: 263 - DNA, 15 bp, Artificial sequence
  Synthetic nucleotides for probe
tagcgcctatacggc

SEQ ID NO: 264 - DNA, 15 bp, Artificial sequence
  Synthetic nucleotides for probe
tgcgcgaatggttac

SEQ ID NO: 265 - DNA, 15 bp, Artificial sequence
  Synthetic nucleotides for probe
tactggccggataat

SEQ ID NO: 266 - DNA, 15 bp, Artificial sequence
  Synthetic nucleotides for probe
ttatacacgatgacg

SEQ ID NO: 267 - DNA, 15 bp, Artificial sequence
  Synthetic nucleotides for probe
accttacgacgacca

SEQ ID NO: 268 - DNA, 15 bp, Artificial sequence
  Synthetic nucleotides for probe
ttagtacagctaccg

SEQ ID NO: 269 - DNA, 15 bp, Artificial sequence
  Synthetic nucleotides for probe
ataagactacggcag

SEQ ID NO: 270 - DNA, 15 bp, Artificial sequence
  Synthetic nucleotides for probe
taggtgatagttcga

SEQ ID NO: 271 - DNA, 15 bp, Artificial sequence
  Synthetic nucleotides for probe
ttatcaattcgccga

SEQ ID NO: 272 - DNA, 15 bp, Artificial sequence
  Synthetic nucleotides for probe
accgtcgcaccttat

SEQ ID NO: 273 - DNA, 15 bp, Artificial sequence
  Synthetic nucleotides for probe
accaatagcgtaccg

SEQ ID NO: 274 - DNA, 15 bp, Artificial sequence
  Synthetic nucleotides for probe
tacgagtgaccggct

SEQ ID NO: 275 - DNA, 15 bp, Artificial sequence
  Synthetic nucleotides for probe
attgccgtcagacta

SEQ ID NO: 276 - DNA, 15 bp, Artificial sequence
  Synthetic nucleotides for probe
tgtcgaaccattcgg

SEQ ID NO: 277 - DNA, 15 bp, Artificial sequence
  Synthetic nucleotides for probe
tcgccttacgtcacg

SEQ ID NO: 278 - DNA, 15 bp, Artificial sequence
  Synthetic nucleotides for probe
agccgactaattccg

SEQ ID NO: 279 - DNA, 15 bp, Artificial sequence
  Synthetic nucleotides for probe
tgtcggtactacgcg

SEQ ID NO: 280 - DNA, 15 bp, Artificial sequence
  Synthetic nucleotides for probe
tagacgtgtaaccga

SEQ ID NO: 281 - DNA, 15 bp, Artificial sequence
  Synthetic nucleotides for probe
aatcgtcaatcgaca

SEQ ID NO: 282 - DNA, 15 bp, Artificial sequence
  Synthetic nucleotides for probe
ttagattctgtcgcg

SEQ ID NO: 283 - DNA, 15 bp, Artificial sequence
  Synthetic nucleotides for probe
tagcactacgcgatt

SEQ ID NO: 284 - DNA, 15 bp, Artificial sequence
  Synthetic nucleotides for probe
acgctgtgagtcgga

SEQ ID NO: 285 - DNA, 15 bp, Artificial sequence
  Synthetic nucleotides for probe
acgataggcgaccat

SEQ ID NO: 286 - DNA, 15 bp, Artificial sequence
  Synthetic nucleotides for probe
tcggcgcttaaccga

SEQ ID NO: 287 - DNA, 15 bp, Artificial sequence
  Synthetic nucleotides for probe
tcgtcggccggtata

SEQ ID NO: 288 - DNA, 15 bp, Artificial sequence
  Synthetic nucleotides for probe
acgatatcttagcga

SEQ ID NO: 289 - DNA, 15 bp, Artificial sequence
  Synthetic nucleotides for probe
tagcggataattcgc

SEQ ID NO: 290 - DNA, 15 bp, Artificial sequence
  Synthetic nucleotides for probe
attccgattgatccg

SEQ ID NO: 291 - DNA, 15 bp, Artificial sequence
  Synthetic nucleotides for probe
agcgcatcctatgcg

SEQ ID NO: 292 - DNA, 15 bp, Artificial sequence
  Synthetic nucleotides for probe
actatgcgttcggtc

SEQ ID NO: 293 - DNA, 15 bp, Artificial sequence
  Synthetic nucleotides for probe
aacgtgtcgtcacgt

SEQ ID NO: 294 - DNA, 15 bp, Artificial sequence
  Synthetic nucleotides for probe
tacttcgctaacgtt

SEQ ID NO: 295 - DNA, 15 bp, Artificial sequence
  Synthetic nucleotides for probe
tctatacgtagaccg

SEQ ID NO: 296 - DNA, 15 bp, Artificial sequence
  Synthetic nucleotides for probe
accgttatgtactcg

SEQ ID NO: 297 - DNA, 15 bp, Artificial sequence
  Synthetic nucleotides for probe
actcgtcaactcgct

SEQ ID NO: 298 - DNA, 15 bp, Artificial sequence
  Synthetic nucleotides for probe
tcgtcgtgcctatac

SEQ ID NO: 299 - DNA, 15 bp, Artificial sequence
  Synthetic nucleotides for probe
acgtaccgattacgt

SEQ ID NO: 300 - DNA, 15 bp, Artificial sequence
  Synthetic nucleotides for probe
acgtcaatccgtata

SEQ ID NO: 301 - DNA, 15 bp, Artificial sequence
  Synthetic nucleotides for probe
tatgcggcactagcc

SEQ ID NO: 302 - DNA, 15 bp, Artificial sequence
  Synthetic nucleotides for probe
atagtcgttaggctc

SEQ ID NO: 303 - DNA, 15 bp, Artificial sequence
  Synthetic nucleotides for probe
taccgagttgcgtac

SEQ ID NO: 304 - DNA, 15 bp, Artificial sequence
  Synthetic nucleotides for probe
atagtatggccgtaa

SEQ ID NO: 305 - DNA, 15 bp, Artificial sequence
  Synthetic nucleotides for probe
tatacggttccgtac

SEQ ID NO: 306 - DNA, 15 bp, Artificial sequence
  Synthetic nucleotides for probe
actagtgcgctaatt

SEQ ID NO: 307 - DNA, 15 bp, Artificial sequence
  Synthetic nucleotides for probe
tcgtccatgcgtata

SEQ ID NO: 308 - DNA, 15 bp, Artificial sequence
  Synthetic nucleotides for probe
atgtcgcgtgaaggt

SEQ ID NO: 309 - DNA, 15 bp, Artificial sequence
  Synthetic nucleotides for probe
acgatatgtatcggt

SEQ ID NO: 310 - DNA, 15 bp, Artificial sequence
  Synthetic nucleotides for probe
tggtcgatctacgca

SEQ ID NO: 311 - DNA, 15 bp, Artificial sequence
  Synthetic nucleotides for probe
aagaccgtcgtattg

SEQ ID NO: 312 - DNA, 15 bp, Artificial sequence
  Synthetic nucleotides for probe
acgtacgcttagatg

SEQ ID NO: 313 - DNA, 15 bp, Artificial sequence
  Synthetic nucleotides for probe
tccgtacgtcgaatc

SEQ ID NO: 314 - DNA, 15 bp, Artificial sequence
  Synthetic nucleotides for probe
tccgcgcactataca

SEQ ID NO: 315 - DNA, 15 bp, Artificial sequence
  Synthetic nucleotides for probe
acggatgttagacgt

SEQ ID NO: 316 - DNA, 15 bp, Artificial sequence
  Synthetic nucleotides for probe
aacgaactgtcaacg

SEQ ID NO: 317 - DNA, 15 bp, Artificial sequence
  Synthetic nucleotides for probe
aacagcgtatgtcgc

SEQ ID NO: 318 - DNA, 15 bp, Artificial sequence
  Synthetic nucleotides for probe
aggacggagcgttat

SEQ ID NO: 319 - DNA, 15 bp, Artificial sequence
  Synthetic nucleotides for probe
tgcacgcaatacggc

SEQ ID NO: 320 - DNA, 15 bp, Artificial sequence
  Synthetic nucleotides for probe
tacaagcgccgattg

SEQ ID NO: 321 - DNA, 15 bp, Artificial sequence
  Synthetic nucleotides for probe
atccaacgcgccata

SEQ ID NO: 322 - DNA, 15 bp, Artificial sequence
  Synthetic nucleotides for probe
attcggttcattgcg

SEQ ID NO: 323 - DNA, 15 bp, Artificial sequence
  Synthetic nucleotides for probe
tattatgtacgtcgg

SEQ ID NO: 324 - DNA, 15 bp, Artificial sequence
  Synthetic nucleotides for probe
tcgaggcgatacgga

SEQ ID NO: 325 - DNA, 15 bp, Artificial sequence
  Synthetic nucleotides for probe
ttgccggcctacgta

SEQ ID NO: 326 - DNA, 15 bp, Artificial sequence
  Synthetic nucleotides for probe
tcgtgtgcgttacat

SEQ ID NO: 327 - DNA, 15 bp, Artificial sequence
  Synthetic nucleotides for probe
accgttgctcgtacg

SEQ ID NO: 328 - DNA, 15 bp, Artificial sequence
  Synthetic nucleotides for probe
tactgatcgtcctat

SEQ ID NO: 329 - DNA, 15 bp, Artificial sequence
  Synthetic nucleotides for probe
tacgattgagttcgg

SEQ ID NO: 330 - DNA, 15 bp, Artificial sequence
  Synthetic nucleotides for probe
atcgtcgaaccgtat

SEQ ID NO: 331 - DNA, 15 bp, Artificial sequence
  Synthetic nucleotides for probe
atagtccgtatctag

SEQ ID NO: 332 - DNA, 15 bp, Artificial sequence
  Synthetic nucleotides for probe
ttgaaccgcactcaa

SEQ ID NO: 333 - DNA, 15 bp, Artificial sequence
  Synthetic nucleotides for probe
ttacgttaaccgttc

SEQ ID NO: 334 - DNA, 15 bp, Artificial sequence
  Synthetic nucleotides for probe
tcatacgaccggcaa

SEQ ID NO: 335 - DNA, 15 bp, Artificial sequence
  Synthetic nucleotides for probe
tatacgcctcgagat

SEQ ID NO: 336 - DNA, 15 bp, Artificial sequence
  Synthetic nucleotides for probe
ttcgcacgatagtac

SEQ ID NO: 337 - DNA, 15 bp, Artificial sequence
  Synthetic nucleotides for probe
acgcagttacggtag

SEQ ID NO: 338 - DNA, 15 bp, Artificial sequence
  Synthetic nucleotides for probe
tcgacgcggtatcga

SEQ ID NO: 339 - DNA, 15 bp, Artificial sequence
  Synthetic nucleotides for probe
atgatcgctcttagt

SEQ ID NO: 340 - DNA, 15 bp, Artificial sequence
  Synthetic nucleotides for probe
tacgacgtaggcact

SEQ ID NO: 341 - DNA, 15 bp, Artificial sequence
  Synthetic nucleotides for probe
ttggtcgtcacaacg

SEQ ID NO: 342 - DNA, 15 bp, Artificial sequence
  Synthetic nucleotides for probe
tagtgcaagtcgcgt

SEQ ID NO: 343 - DNA, 15 bp, Artificial sequence
  Synthetic nucleotides for probe
tcacggtacatcgat

SEQ ID NO: 344 - DNA, 15 bp, Artificial sequence
  Synthetic nucleotides for probe
atccattattcggcg

SEQ ID NO: 345 - DNA, 15 bp, Artificial sequence
  Synthetic nucleotides for probe
acgtgttcattcgga

SEQ ID NO: 346 - DNA, 15 bp, Artificial sequence
  Synthetic nucleotides for probe
tactcgcgttaacgt

SEQ ID NO: 347 - DNA, 15 bp, Artificial sequence
  Synthetic nucleotides for probe
ttagagtagtcgccg

SEQ ID NO: 348 - DNA, 15 bp, Artificial sequence
  Synthetic nucleotides for probe
ataggtagtcgcctt

SEQ ID NO: 349 - DNA, 15 bp, Artificial sequence
  Synthetic nucleotides for probe
atagtcgcgcgttgc

SEQ ID NO: 350 - DNA, 15 bp, Artificial sequence
  Synthetic nucleotides for probe
tacgcacactaacga

SEQ ID NO: 351 - DNA, 15 bp, Artificial sequence
  Synthetic nucleotides for probe
aactataactcgcga

SEQ ID NO: 352 - DNA, 15 bp, Artificial sequence
  Synthetic nucleotides for probe
attatattgtccgcg

SEQ ID NO: 353 - DNA, 15 bp, Artificial sequence
  Synthetic nucleotides for probe
tcgtgtatgcgaacc

SEQ ID NO: 354 - DNA, 15 bp, Artificial sequence
  Synthetic nucleotides for probe
atacgagtagcgccg

SEQ ID NO: 355 - DNA, 15 bp, Artificial sequence
  Synthetic nucleotides for probe
tatcggctatcgctc

SEQ ID NO: 356 - DNA, 15 bp, Artificial sequence
  Synthetic nucleotides for probe
tagtcatagctcgcc

SEQ ID NO: 357 - DNA, 15 bp, Artificial sequence
  Synthetic nucleotides for probe
atcaccgattcgtgc

SEQ ID NO: 358 - DNA, 15 bp, Artificial sequence
  Synthetic nucleotides for probe
tgttctcgcgtatgg

SEQ ID NO: 359 - DNA, 15 bp, Artificial sequence
  Synthetic nucleotides for probe
tccaacgtatcgtcc

SEQ ID NO: 360 - DNA, 15 bp, Artificial sequence
  Synthetic nucleotides for probe
ttcgcgtccattcgc

SEQ ID NO: 361 - DNA, 15 bp, Artificial sequence
  Synthetic nucleotides for probe
agcgtgctcgactta

SEQ ID NO: 362 - DNA, 15 bp, Artificial sequence
  Synthetic nucleotides for probe
attacgctgttagcg

SEQ ID NO: 363 - DNA, 15 bp, Artificial sequence
  Synthetic nucleotides for probe
taggtacaatcgcgg

SEQ ID NO: 364 - DNA, 15 bp, Artificial sequence
  Synthetic nucleotides for probe
tgatctatcgaacga

SEQ ID NO: 365 - DNA, 15 bp, Artificial sequence
  Synthetic nucleotides for probe
tcgattgcgacgcaa

SEQ ID NO: 366 - DNA, 15 bp, Artificial sequence
  Synthetic nucleotides for probe
ttgcgctatccgtga

SEQ ID NO: 367 - DNA, 15 bp, Artificial sequence
  Synthetic nucleotides for probe
tcgaggatagcgtat

SEQ ID NO: 368 - DNA, 15 bp, Artificial sequence
  Synthetic nucleotides for probe
aagacgcaacctcgt

SEQ ID NO: 369 - DNA, 15 bp, Artificial sequence
  Synthetic nucleotides for probe
tcgctatacgaatct

SEQ ID NO: 370 - DNA, 15 bp, Artificial sequence
  Synthetic nucleotides for probe
ttagcggttcactcg

SEQ ID NO: 371 - DNA, 15 bp, Artificial sequence
  Synthetic nucleotides for probe
tatacgatacttgcg

SEQ ID NO: 372 - DNA, 15 bp, Artificial sequence
  Synthetic nucleotides for probe
taagcatgcgattac

SEQ ID NO: 373 - DNA, 15 bp, Artificial sequence
  Synthetic nucleotides for probe
tcgatcgagttacaa

SEQ ID NO: 374 - DNA, 15 bp, Artificial sequence
  Synthetic nucleotides for probe
agttagtcgcgccaa

SEQ ID NO: 375 - DNA, 15 bp, Artificial sequence
  Synthetic nucleotides for probe
aggcggaccgatcaa

SEQ ID NO: 376 - DNA, 15 bp, Artificial sequence
  Synthetic nucleotides for probe
agtattcggctcgtg

SEQ ID NO: 377 - DNA, 15 bp, Artificial sequence
  Synthetic nucleotides for probe
aagtcgtgatccgtc

SEQ ID NO: 378 - DNA, 15 bp, Artificial sequence
  Synthetic nucleotides for probe
ttgtgttacgtccgc

SEQ ID NO: 379 - DNA, 15 bp, Artificial sequence
  Synthetic nucleotides for probe
ttccatacgagtgcg

SEQ ID NO: 380 - DNA, 15 bp, Artificial sequence
  Synthetic nucleotides for probe
agactcgtacattag

SEQ ID NO: 381 - DNA, 15 bp, Artificial sequence
  Synthetic nucleotides for probe
tagtatctccgatca

SEQ ID NO: 382 - DNA, 15 bp, Artificial sequence
  Synthetic nucleotides for probe
acggtcgtgcttcta

SEQ ID NO: 383 - DNA, 15 bp, Artificial sequence
  Synthetic nucleotides for probe
atcggacgtaagtcc

SEQ ID NO: 384 - DNA, 15 bp, Artificial sequence
  Synthetic nucleotides for probe
aacagtacgctacgt

SEQ ID NO: 385 - DNA, 15 bp, Artificial sequence
  Synthetic nucleotides for probe
taccgctcgcgtaac

SEQ ID NO: 386 - DNA, 15 bp, Artificial sequence
  Synthetic nucleotides for probe
aggtacgtaaccgcg

SEQ ID NO: 387 - DNA, 15 bp, Artificial sequence
  Synthetic nucleotides for probe
acgtacggcctgtgt

SEQ ID NO: 388 - DNA, 15 bp, Artificial sequence
  Synthetic nucleotides for probe
accgtcgttattagg

SEQ ID NO: 389 - DNA, 15 bp, Artificial sequence
  Synthetic nucleotides for probe
tcggtccgcatatcg

SEQ ID NO: 390 - DNA, 15 bp, Artificial sequence
  Synthetic nucleotides for probe
atccgacgatcgaga

SEQ ID NO: 391 - DNA, 15 bp, Artificial sequence
  Synthetic nucleotides for probe
tcgaacgcatcagac

SEQ ID NO: 392 - DNA, 15 bp, Artificial sequence
  Synthetic nucleotides for probe
tcgctcgtataggct

SEQ ID NO: 393 - DNA, 15 bp, Artificial sequence
  Synthetic nucleotides for probe
tatgaggcctagtcg

SEQ ID NO: 394 - DNA, 15 bp, Artificial sequence
  Synthetic nucleotides for probe
tagtcgctattcggc

SEQ ID NO: 395 - DNA, 15 bp, Artificial sequence
  Synthetic nucleotides for probe
taatctaccgctagt

SEQ ID NO: 396 - DNA, 15 bp, Artificial sequence
  Synthetic nucleotides for probe
ttcgaacaacgcgct

SEQ ID NO: 397 - DNA, 15 bp, Artificial sequence
  Synthetic nucleotides for probe
acgtgcgttagcttc

SEQ ID NO: 398 - DNA, 15 bp, Artificial sequence
  Synthetic nucleotides for probe
agttaatcgcggtcc

SEQ ID NO: 399 - DNA, 15 bp, Artificial sequence
  Synthetic nucleotides for probe
ttattaggtctcgtc

SEQ ID NO: 400 - DNA, 15 bp, Artificial sequence
  Synthetic nucleotides for probe
atcgttacggcgtag

SEQ ID NO: 401 - DNA, 15 bp, Artificial sequence
  Synthetic nucleotides for probe
attacggtagaacgc

SEQ ID NO: 402 - DNA, 15 bp, Artificial sequence
  Synthetic nucleotides for probe
tactactgccgtgcg

SEQ ID NO: 403 - DNA, 15 bp, Artificial sequence
  Synthetic nucleotides for probe
ataggtaacgaccgt

SEQ ID NO: 404 - DNA, 15 bp, Artificial sequence
  Synthetic nucleotides for probe
tagacgtaatcggac

SEQ ID NO: 405 - DNA, 15 bp, Artificial sequence
  Synthetic nucleotides for probe
taggtaccgatcgag

SEQ ID NO: 406 - DNA, 15 bp, Artificial sequence
  Synthetic nucleotides for probe
ttaacgacgctagac

SEQ ID NO: 407 - DNA, 15 bp, Artificial sequence
  Synthetic nucleotides for probe
tagccgacgcaagtg

SEQ ID NO: 408 - DNA, 15 bp, Artificial sequence
  Synthetic nucleotides for probe
tacggttgaatctac

SEQ ID NO: 409 - DNA, 15 bp, Artificial sequence
  Synthetic nucleotides for probe
atggcgatagcgtcg

SEQ ID NO: 410 - DNA, 15 bp, Artificial sequence
  Synthetic nucleotides for probe
tgttacgcgtccaga

SEQ ID NO: 411 - DNA, 15 bp, Artificial sequence
  Synthetic nucleotides for probe
atcattcgcgttcgc

SEQ ID NO: 412 - DNA, 15 bp, Artificial sequence
  Synthetic nucleotides for probe
actacggacgttcga

SEQ ID NO: 413 - DNA, 15 bp, Artificial sequence
  Synthetic nucleotides for probe
tcgctaacataacga

SEQ ID NO: 414 - DNA, 15 bp, Artificial sequence
  Synthetic nucleotides for probe
acgatatgagtgaac

SEQ ID NO: 415 - DNA, 15 bp, Artificial sequence
  Synthetic nucleotides for probe
ttgcgttccgatacg

SEQ ID NO: 416 - DNA, 15 bp, Artificial sequence
  Synthetic nucleotides for probe
tagtagtgccggcgt

SEQ ID NO: 417 - DNA, 15 bp, Artificial sequence
  Synthetic nucleotides for probe
ttaacgcgtcgtacg

SEQ ID NO: 418 - DNA, 15 bp, Artificial sequence
  Synthetic nucleotides for probe
tccaacggtcattcg

SEQ ID NO: 419 - DNA, 15 bp, Artificial sequence
  Synthetic nucleotides for probe
tatgatatggcgtgc

SEQ ID NO: 420 - DNA, 15 bp, Artificial sequence
  Synthetic nucleotides for probe
tatccgtagtacgct

SEQ ID NO: 421 - DNA, 15 bp, Artificial sequence
  Synthetic nucleotides for probe
acacgttatgtcgcg

SEQ ID NO: 422 - DNA, 15 bp, Artificial sequence
  Synthetic nucleotides for probe
acgctcatcgcgatt

SEQ ID NO: 423 - DNA, 15 bp, Artificial sequence
  Synthetic nucleotides for probe
accggagtaggtata

SEQ ID NO: 424 - DNA, 15 bp, Artificial sequence
  Synthetic nucleotides for probe
ttacgaatcgtgcac

SEQ ID NO: 425 - DNA, 15 bp, Artificial sequence
  Synthetic nucleotides for probe
ttgaacgctattacg

SEQ ID NO: 426 - DNA, 15 bp, Artificial sequence
  Synthetic nucleotides for probe
tactatatccgcgaa

SEQ ID NO: 427 - DNA, 15 bp, Artificial sequence
  Synthetic nucleotides for probe
tcgagctattcggta

SEQ ID NO: 428 - DNA, 15 bp, Artificial sequence
  Synthetic nucleotides for probe
tactagtcgttacac

SEQ ID NO: 429 - DNA, 15 bp, Artificial sequence
  Synthetic nucleotides for probe
taggtcgcgtaccgt

SEQ ID NO: 430 - DNA, 15 bp, Artificial sequence
  Synthetic nucleotides for probe
ttcgcgttctatcta

SEQ ID NO: 431 - DNA, 15 bp, Artificial sequence
  Synthetic nucleotides for probe
tcgcggcgttgttag

SEQ ID NO: 432 - DNA, 15 bp, Artificial sequence
  Synthetic nucleotides for probe
actatagcgcgcttg

SEQ ID NO: 433 - DNA, 15 bp, Artificial sequence
  Synthetic nucleotides for probe
tacgatcaagtcgta

SEQ ID NO: 434 - DNA, 15 bp, Artificial sequence
  Synthetic nucleotides for probe
taatcgtcgcaactg

SEQ ID NO: 435 - DNA, 15 bp, Artificial sequence
  Synthetic nucleotides for probe
aagtaggcgagtcgt

SEQ ID NO: 436 - DNA, 15 bp, Artificial sequence
  Synthetic nucleotides for probe
tacgatccggtatgt

SEQ ID NO: 437 - DNA, 15 bp, Artificial sequence
  Synthetic nucleotides for probe
tatgatccgacgcct

SEQ ID NO: 438 - DNA, 15 bp, Artificial sequence
  Synthetic nucleotides for probe
tagattcgtgtctcg

SEQ ID NO: 439 - DNA, 15 bp, Artificial sequence
  Synthetic nucleotides for probe
ttaggcgcgcttaag

SEQ ID NO: 440 - DNA, 15 bp, Artificial sequence
  Synthetic nucleotides for probe
acggctagtagtgac

SEQ ID NO: 441 - DNA, 15 bp, Artificial sequence
  Synthetic nucleotides for probe
agcgctattaaggcc

SEQ ID NO: 442 - DNA, 15 bp, Artificial sequence
  Synthetic nucleotides for probe
tacgaggtaactatc

SEQ ID NO: 443 - DNA, 15 bp, Artificial sequence
  Synthetic nucleotides for probe
aggtagttcgtgccg

SEQ ID NO: 444 - DNA, 15 bp, Artificial sequence
  Synthetic nucleotides for probe
tccgtagaacgatta

SEQ ID NO: 445 - DNA, 15 bp, Artificial sequence
  Synthetic nucleotides for probe
tcgtgaacgcactaa

SEQ ID NO: 446 - DNA, 15 bp, Artificial sequence
  Synthetic nucleotides for probe
atagatcatcggccg

SEQ ID NO: 447 - DNA, 15 bp, Artificial sequence
  Synthetic nucleotides for probe
tctaccggtcgatcg

SEQ ID NO: 448 - DNA, 15 bp, Artificial sequence
  Synthetic nucleotides for probe
tattcggtcgttccg

SEQ ID NO: 449 - DNA, 15 bp, Artificial sequence
  Synthetic nucleotides for probe
agcgtacgcatccgt

SEQ ID NO: 450 - DNA, 15 bp, Artificial sequence
  Synthetic nucleotides for probe
acgcattgcacaatt

SEQ ID NO: 451 - DNA, 15 bp, Artificial sequence
  Synthetic nucleotides for probe
ttaagttacgtcgcc

SEQ ID NO: 452 - DNA, 15 bp, Artificial sequence
  Synthetic nucleotides for probe
acgattcatagcacc

SEQ ID NO: 453 - DNA, 15 bp, Artificial sequence
  Synthetic nucleotides for probe
actagtcacgacgaa

SEQ ID NO: 454 - DNA, 15 bp, Artificial sequence
  Synthetic nucleotides for probe
acctcacttagtcga

SEQ ID NO: 455 - DNA, 15 bp, Artificial sequence
  Synthetic nucleotides for probe
aactagcgcagcgta

SEQ ID NO: 456 - DNA, 15 bp, Artificial sequence
  Synthetic nucleotides for probe
aacgcgaagtaagcg

SEQ ID NO: 457 - DNA, 15 bp, Artificial sequence
  Synthetic nucleotides for probe
aacgcgactagctcg

SEQ ID NO: 458 - DNA, 15 bp, Artificial sequence
  Synthetic nucleotides for probe
atacgggatttgcgt

SEQ ID NO: 459 - DNA, 15 bp, Artificial sequence
  Synthetic nucleotides for probe
tgcgtccaatttcga

SEQ ID NO: 460 - DNA, 15 bp, Artificial sequence
  Synthetic nucleotides for probe
tcgtgttacgttggg

SEQ ID NO: 461 - DNA, 15 bp, Artificial sequence
  Synthetic nucleotides for probe
tttattcgtcccgat

SEQ ID NO: 462 - DNA, 15 bp, Artificial sequence
  Synthetic nucleotides for probe
taccattcggcccga

SEQ ID NO: 463 - DNA, 15 bp, Artificial sequence
  Synthetic nucleotides for probe
atgactaaacgcgcc

SEQ ID NO: 464 - DNA, 15 bp, Artificial sequence
  Synthetic nucleotides for probe
aatcccattgcgacg

SEQ ID NO: 465 - DNA, 15 bp, Artificial sequence
  Synthetic nucleotides for probe
agcgatactcccgaa

SEQ ID NO: 466 - DNA, 15 bp, Artificial sequence
  Synthetic nucleotides for probe
atcagtgcgtttacg

SEQ ID NO: 467 - DNA, 15 bp, Artificial sequence
  Synthetic nucleotides for probe
tgacccgagtttcgt

SEQ ID NO: 468 - DNA, 15 bp, Artificial sequence
  Synthetic nucleotides for probe
acgacgcggaaactt

SEQ ID NO: 469 - DNA, 15 bp, Artificial sequence
  Synthetic nucleotides for probe
actaaacgaaacgtg

SEQ ID NO: 470 - DNA, 15 bp, Artificial sequence
  Synthetic nucleotides for probe
atcggaccgtaaact

SEQ ID NO: 471 - DNA, 15 bp, Artificial sequence
  Synthetic nucleotides for probe
tagggtcccgctata

SEQ ID NO: 472 - DNA, 15 bp, Artificial sequence
  Synthetic nucleotides for probe
tcgtaaacgggactg

SEQ ID NO: 473 - DNA, 15 bp, Artificial sequence
  Synthetic nucleotides for probe
tcccttactcgctac

SEQ ID NO: 474 - DNA, 15 bp, Artificial sequence
  Synthetic nucleotides for probe
taaagcgcatacgac

SEQ ID NO: 475 - DNA, 15 bp, Artificial sequence
  Synthetic nucleotides for probe
aatccgcgcataaag

SEQ ID NO: 476 - DNA, 15 bp, Artificial sequence
  Synthetic nucleotides for probe
aatcatgcgtttccg

SEQ ID NO: 477 - DNA, 15 bp, Artificial sequence
  Synthetic nucleotides for probe
tcgatttgcgtccga

SEQ ID NO: 478 - DNA, 15 bp, Artificial sequence
  Synthetic nucleotides for probe
tgagacgccgattta

SEQ ID NO: 479 - DNA, 15 bp, Artificial sequence
  Synthetic nucleotides for probe
tatcaaatacgtcgc

SEQ ID NO: 480 - DNA, 15 bp, Artificial sequence
  Synthetic nucleotides for probe
tcgcgctttcatacg

SEQ ID NO: 481 - DNA, 15 bp, Artificial sequence
  Synthetic nucleotides for probe
agtgcgtaaagcgcc

SEQ ID NO: 482 - DNA, 15 bp, Artificial sequence
  Synthetic nucleotides for probe
tcgctataaaggtcc

SEQ ID NO: 483 - DNA, 15 bp, Artificial sequence
  Synthetic nucleotides for probe
atacccgtgttaacg

SEQ ID NO: 484 - DNA, 15 bp, Artificial sequence
  Synthetic nucleotides for probe
acggcaattagggtt

SEQ ID NO: 485 - DNA, 15 bp, Artificial sequence
  Synthetic nucleotides for probe
taaattgccgggagt

SEQ ID NO: 486 - DNA, 15 bp, Artificial sequence
  Synthetic nucleotides for probe
aacgagatcgtaccc

SEQ ID NO: 487 - DNA, 15 bp, Artificial sequence
  Synthetic nucleotides for probe
tacgtaaactcgtgc

SEQ ID NO: 488 - DNA, 15 bp, Artificial sequence
  Synthetic nucleotides for probe
aacgcggtttgctac

SEQ ID NO: 489 - DNA, 15 bp, Artificial sequence
  Synthetic nucleotides for probe
acgcacgatcgtttc

SEQ ID NO: 490 - DNA, 15 bp, Artificial sequence
  Synthetic nucleotides for probe
aatttcgacgtagag

SEQ ID NO: 491 - DNA, 15 bp, Artificial sequence
  Synthetic nucleotides for probe
tatcgcgggcgaaat

SEQ ID NO: 492 - DNA, 15 bp, Artificial sequence
  Synthetic nucleotides for probe
tccgtaaacgttacg

SEQ ID NO: 493 - DNA, 15 bp, Artificial sequence
  Synthetic nucleotides for probe
tattaacccgaccac

SEQ ID NO: 494 - DNA, 15 bp, Artificial sequence
  Synthetic nucleotides for probe
taccctgtacgcacg

SEQ ID NO: 495 - DNA, 15 bp, Artificial sequence
  Synthetic nucleotides for probe
aagtcccgcgtaaat

SEQ ID NO: 496 - DNA, 15 bp, Artificial sequence
  Synthetic nucleotides for probe
tcccgctattcaggt

SEQ ID NO: 497 - DNA, 15 bp, Artificial sequence
  Synthetic nucleotides for probe
tctaaaccgcttacg

SEQ ID NO: 498 - DNA, 15 bp, Artificial sequence
  Synthetic nucleotides for probe
ttgcgaacgcaattt

SEQ ID NO: 499 - DNA, 15 bp, Artificial sequence
  Synthetic nucleotides for probe
tgatagcggtttggc

SEQ ID NO: 500 - DNA, 15 bp, Artificial sequence
  Synthetic nucleotides for probe
tcaacccgtcgttag

SEQ ID NO: 501 - DNA, 15 bp, Artificial sequence
  Synthetic nucleotides for probe
tctacgcaatacccg

SEQ ID NO: 502 - DNA, 15 bp, Artificial sequence
  Synthetic nucleotides for probe
ataaacgctacgctt

SEQ ID NO: 503 - DNA, 15 bp, Artificial sequence
  Synthetic nucleotides for probe
acgtattagtttgcg

SEQ ID NO: 504 - DNA, 15 bp, Artificial sequence
  Synthetic nucleotides for probe
agtacgggcttacca

SEQ ID NO: 505 - DNA, 15 bp, Artificial sequence
  Synthetic nucleotides for probe
accataaagcgagcg

SEQ ID NO: 506 - DNA, 15 bp, Artificial sequence
  Synthetic nucleotides for probe
acgtaacgtgccctt

SEQ ID NO: 507 - DNA, 15 bp, Artificial sequence
  Synthetic nucleotides for probe
atgtatcccgtagtc

SEQ ID NO: 508 - DNA, 15 bp, Artificial sequence
  Synthetic nucleotides for probe
actatcgtttaggcg

SEQ ID NO: 509 - DNA, 15 bp, Artificial sequence
  Synthetic nucleotides for probe
ataacgcgggctact

SEQ ID NO: 510 - DNA, 15 bp, Artificial sequence
  Synthetic nucleotides for probe
taatacggcaacccg

SEQ ID NO: 511 - DNA, 15 bp, Artificial sequence
  Synthetic nucleotides for probe
taaacgcgatcggca

SEQ ID NO: 512 - DNA, 15 bp, Artificial sequence
  Synthetic nucleotides for probe
tttctactaccgtcg

SEQ ID NO: 513 - DNA, 15 bp, Artificial sequence
  Synthetic nucleotides for probe
tttcgcacgggttac

SEQ ID NO: 514 - DNA, 15 bp, Artificial sequence
  Synthetic nucleotides for probe
tggctacgaacgaaa

SEQ ID NO: 515 - DNA, 15 bp, Artificial sequence
  Synthetic nucleotides for probe
tttgcgcgggtaaca

SEQ ID NO: 516 - DNA, 15 bp, Artificial sequence
  Synthetic nucleotides for probe
agcgcgaaatcgaca

SEQ ID NO: 517 - DNA, 15 bp, Artificial sequence
  Synthetic nucleotides for probe
acccgttaagaacgg

SEQ ID NO: 518 - DNA, 15 bp, Artificial sequence
  Synthetic nucleotides for probe
aacgggctagaatcg

SEQ ID NO: 519 - DNA, 15 bp, Artificial sequence
  Synthetic nucleotides for probe
accggtcccgattta

SEQ ID NO: 520 - DNA, 15 bp, Artificial sequence
  Synthetic nucleotides for probe
tatcaacccgacgcc

SEQ ID NO: 521 - DNA, 15 bp, Artificial sequence
  Synthetic nucleotides for probe
tcgcggattaaatag

SEQ ID NO: 522 - DNA, 15 bp, Artificial sequence
  Synthetic nucleotides for probe
tttggtgcttcgcgg

SEQ ID NO: 523 - DNA, 15 bp, Artificial sequence
  Synthetic nucleotides for probe
aaagtattcgcgaac

SEQ ID NO: 524 - DNA, 15 bp, Artificial sequence
  Synthetic nucleotides for probe
tagacgaacctttcg

SEQ ID NO: 525 - DNA, 15 bp, Artificial sequence
  Synthetic nucleotides for probe
aaatcggtatgcgct

SEQ ID NO: 526 - DNA, 15 bp, Artificial sequence
  Synthetic nucleotides for probe
tcgacgcgagaaact

SEQ ID NO: 527 - DNA, 15 bp, Artificial sequence
  Synthetic nucleotides for probe
ttaagtcgggcaata

SEQ ID NO: 528 - DNA, 15 bp, Artificial sequence
  Synthetic nucleotides for probe
tcggatataaagacg

SEQ ID NO: 529 - DNA, 15 bp, Artificial sequence
  Synthetic nucleotides for probe
ataaagtgtcggtcg

SEQ ID NO: 530 - DNA, 15 bp, Artificial sequence
  Synthetic nucleotides for probe
taaactcgtatcccg

SEQ ID NO: 531 - DNA, 15 bp, Artificial sequence
  Synthetic nucleotides for probe
aaatccgtgacgtac

SEQ ID NO: 532 - DNA, 15 bp, Artificial sequence
  Synthetic nucleotides for probe
acatctaacgggcgt

SEQ ID NO: 533 - DNA, 15 bp, Artificial sequence
  Synthetic nucleotides for probe
tcgtaccctatagtt

SEQ ID NO: 534 - DNA, 15 bp, Artificial sequence
  Synthetic nucleotides for probe
agcgtctaaacggac

SEQ ID NO: 535 - DNA, 15 bp, Artificial sequence
  Synthetic nucleotides for probe
acgtatgctttcggg

SEQ ID NO: 536 - DNA, 15 bp, Artificial sequence
  Synthetic nucleotides for probe
tcgattagggtgcct

SEQ ID NO: 537 - DNA, 15 bp, Artificial sequence
  Synthetic nucleotides for probe
attcccgcttaagat

SEQ ID NO: 538 - DNA, 15 bp, Artificial sequence
  Synthetic nucleotides for probe
accgtaatcgggcca

SEQ ID NO: 539 - DNA, 15 bp, Artificial sequence
  Synthetic nucleotides for probe
tcgtttcgtcgtacc

SEQ ID NO: 540 - DNA, 15 bp, Artificial sequence
  Synthetic nucleotides for probe
tcgatcgggttagct

SEQ ID NO: 541 - DNA, 15 bp, Artificial sequence
  Synthetic nucleotides for probe
tgtacgcccaatcgc

SEQ ID NO: 542 - DNA, 15 bp, Artificial sequence
  Synthetic nucleotides for probe
acggcccgacattta

SEQ ID NO: 543 - DNA, 15 bp, Artificial sequence
  Synthetic nucleotides for probe
ttcggtaaataccga

SEQ ID NO: 544 - DNA, 15 bp, Artificial sequence
  Synthetic nucleotides for probe
agggaatatacgacg

SEQ ID NO: 545 - DNA, 15 bp, Artificial sequence
  Synthetic nucleotides for probe
tgacgcacctttacg

SEQ ID NO: 546 - DNA, 15 bp, Artificial sequence
  Synthetic nucleotides for probe
tatttgccggacgta

SEQ ID NO: 547 - DNA, 15 bp, Artificial sequence
  Synthetic nucleotides for probe
taaatgccgttccga

SEQ ID NO: 548 - DNA, 15 bp, Artificial sequence
  Synthetic nucleotides for probe
ttaagcgcccatacg

SEQ ID NO: 549 - DNA, 15 bp, Artificial sequence
  Synthetic nucleotides for probe
tttcaaccgcgattc

SEQ ID NO: 550 - DNA, 15 bp, Artificial sequence
  Synthetic nucleotides for probe
aactatccgaacccg

SEQ ID NO: 551 - DNA, 15 bp, Artificial sequence
  Synthetic nucleotides for probe
tttatgcgagctacg

SEQ ID NO: 552 - DNA, 15 bp, Artificial sequence
  Synthetic nucleotides for probe
agtactagcgcgggt

SEQ ID NO: 553 - DNA, 15 bp, Artificial sequence
  Synthetic nucleotides for probe
tttattacgccgaga

SEQ ID NO: 554 - DNA, 15 bp, Artificial sequence
  Synthetic nucleotides for probe
atatatcgggatgcg

SEQ ID NO: 555 - DNA, 15 bp, Artificial sequence
  Synthetic nucleotides for probe
tttaaccggacgata

SEQ ID NO: 556 - DNA, 15 bp, Artificial sequence
  Synthetic nucleotides for probe
taaacgttggtcgta

SEQ ID NO: 557 - DNA, 15 bp, Artificial sequence
  Synthetic nucleotides for probe
tcgatagggtatagt

SEQ ID NO: 558 - DNA, 15 bp, Artificial sequence
  Synthetic nucleotides for probe
tagtaaacctgcgcc

SEQ ID NO: 559 - DNA, 15 bp, Artificial sequence
  Synthetic nucleotides for probe
aagtttcgcgctgac

SEQ ID NO: 560 - DNA, 15 bp, Artificial sequence
  Synthetic nucleotides for probe
tgataaacgtcgcct

SEQ ID NO: 561 - DNA, 15 bp, Artificial sequence
  Synthetic nucleotides for probe
attgaaacgccgtcg

SEQ ID NO: 562 - DNA, 15 bp, Artificial sequence
  Synthetic nucleotides for probe
tcgcgggttgatcaa

SEQ ID NO: 563 - DNA, 15 bp, Artificial sequence
  Synthetic nucleotides for probe
taaatcgacgcgtag

SEQ ID NO: 564 - DNA, 15 bp, Artificial sequence
  Synthetic nucleotides for probe
tttacggtcgtcgcc

SEQ ID NO: 565 - DNA, 15 bp, Artificial sequence
  Synthetic nucleotides for probe
tacgaggaaagttag

SEQ ID NO: 566 - DNA, 15 bp, Artificial sequence
  Synthetic nucleotides for probe
tatttgcgtggtcgg

SEQ ID NO: 567 - DNA, 15 bp, Artificial sequence
  Synthetic nucleotides for probe
ataaagcgtataccc

SEQ ID NO: 568 - DNA, 15 bp, Artificial sequence
  Synthetic nucleotides for probe
taagtcgggtcgaca

SEQ ID NO: 569 - DNA, 15 bp, Artificial sequence
  Synthetic nucleotides for probe
tacgccgggtactta

SEQ ID NO: 570 - DNA, 15 bp, Artificial sequence
  Synthetic nucleotides for probe
agataacccgcgcgt

SEQ ID NO: 571 - DNA, 15 bp, Artificial sequence
  Synthetic nucleotides for probe
acgggtccgtcgatt

SEQ ID NO: 572 - DNA, 15 bp, Artificial sequence
  Synthetic nucleotides for probe
acatgagcgttaccc

SEQ ID NO: 573 - DNA, 15 bp, Artificial sequence
  Synthetic nucleotides for probe
acggcgtataaacct

SEQ ID NO: 574 - DNA, 15 bp, Artificial sequence
  Synthetic nucleotides for probe
acgactaatcgccca

SEQ ID NO: 575 - DNA, 15 bp, Artificial sequence
  Synthetic nucleotides for probe
aaacgctattgccgt

SEQ ID NO: 576 - DNA, 15 bp, Artificial sequence
  Synthetic nucleotides for probe
attatcgaaacggcc

SEQ ID NO: 577 - DNA, 15 bp, Artificial sequence
  Synthetic nucleotides for probe
acgaacaaacatgcg

SEQ ID NO: 578 - DNA, 15 bp, Artificial sequence
  Synthetic nucleotides for probe
tcccgaccgagataa

SEQ ID NO: 579 - DNA, 15 bp, Artificial sequence
  Synthetic nucleotides for probe
tgcgtaaagtgtacg

SEQ ID NO: 580 - DNA, 15 bp, Artificial sequence
  Synthetic nucleotides for probe
tttacggttacccga

SEQ ID NO: 581 - DNA, 15 bp, Artificial sequence
  Synthetic nucleotides for probe
atagactgacgcggg

SEQ ID NO: 582 - DNA, 15 bp, Artificial sequence
  Synthetic nucleotides for probe
atatgcccgtaacgc

SEQ ID NO: 583 - DNA, 15 bp, Artificial sequence
  Synthetic nucleotides for probe
atttagtgttcgccc

SEQ ID NO: 584 - DNA, 15 bp, Artificial sequence
  Synthetic nucleotides for probe
acgcattatgggcgt

SEQ ID NO: 585 - DNA, 15 bp, Artificial sequence
  Synthetic nucleotides for probe
tcgttataggtaccc

SEQ ID NO: 586 - DNA, 15 bp, Artificial sequence
  Synthetic nucleotides for probe
tatcgtaacgcaccc

SEQ ID NO: 587 - DNA, 15 bp, Artificial sequence
  Synthetic nucleotides for probe
acgacgattcccacg

SEQ ID NO: 588 - DNA, 15 bp, Artificial sequence
  Synthetic nucleotides for probe
tttcacgatcgcacc

SEQ ID NO: 589 - DNA, 15 bp, Artificial sequence
  Synthetic nucleotides for probe
tcgacccgcatatag

SEQ ID NO: 590 - DNA, 15 bp, Artificial sequence
  Synthetic nucleotides for probe
acctcggtaacgaaa

SEQ ID NO: 591 - DNA, 15 bp, Artificial sequence
  Synthetic nucleotides for probe
tataagagtcgcggg

SEQ ID NO: 592 - DNA, 15 bp, Artificial sequence
  Synthetic nucleotides for probe
tgggcgaaattctcg

SEQ ID NO: 593 - DNA, 15 bp, Artificial sequence
  Synthetic nucleotides for probe
acgcgctaaattcga

SEQ ID NO: 594 - DNA, 15 bp, Artificial sequence
  Synthetic nucleotides for probe
tttattctatcgcgc

SEQ ID NO: 595 - DNA, 15 bp, Artificial sequence
  Synthetic nucleotides for probe
ttacgattcccgtcg

SEQ ID NO: 596 - DNA, 15 bp, Artificial sequence
  Synthetic nucleotides for probe
atttcgatccgcgat

SEQ ID NO: 597 - DNA, 15 bp, Artificial sequence
  Synthetic nucleotides for probe
tcgtttacgtaccgc

SEQ ID NO: 598 - DNA, 15 bp, Artificial sequence
  Synthetic nucleotides for probe
taacgtaggtcgttt

SEQ ID NO: 599 - DNA, 15 bp, Artificial sequence
  Synthetic nucleotides for probe
atacccgtaagcgag

SEQ ID NO: 600 - DNA, 15 bp, Artificial sequence
  Synthetic nucleotides for probe
taaccgacccggctt

SEQ ID NO: 601 - DNA, 15 bp, Artificial sequence
  Synthetic nucleotides for probe
tacccgccgtaatcc

SEQ ID NO: 602 - DNA, 15 bp, Artificial sequence
  Synthetic nucleotides for probe
acgcggaatttacgt

SEQ ID NO: 603 - DNA, 15 bp, Artificial sequence
  Synthetic nucleotides for probe
acgtaacgggtgatc

SEQ ID NO: 604 - DNA, 15 bp, Artificial sequence
  Synthetic nucleotides for probe
atcgcagttaaacgg

SEQ ID NO: 605 - DNA, 15 bp, Artificial sequence
  Synthetic nucleotides for probe
agaattcgttcgggt

SEQ ID NO: 606 - DNA, 15 bp, Artificial sequence
  Synthetic nucleotides for probe
taggaaatcgcgccg

SEQ ID NO: 607 - DNA, 15 bp, Artificial sequence
  Synthetic nucleotides for probe
taaacgtccctacgc

SEQ ID NO: 608 - DNA, 15 bp, Artificial sequence
  Synthetic nucleotides for probe
atttacgctagatgg

SEQ ID NO: 609 - DNA, 15 bp, Artificial sequence
  Synthetic nucleotides for probe
tactatgggtcgttc

SEQ ID NO: 610 - DNA, 15 bp, Artificial sequence
  Synthetic nucleotides for probe
atcacgatcgatccc

SEQ ID NO: 611 - DNA, 15 bp, Artificial sequence
  Synthetic nucleotides for probe
tcgtttgacgcgtgt

SEQ ID NO: 612 - DNA, 15 bp, Artificial sequence
  Synthetic nucleotides for probe
ttcgcccgaattact

SEQ ID NO: 613 - DNA, 15 bp, Artificial sequence
  Synthetic nucleotides for probe
acgctgcgcgtttat

SEQ ID NO: 614 - DNA, 15 bp, Artificial sequence
  Synthetic nucleotides for probe
ttgagtagacgcccg

SEQ ID NO: 615 - DNA, 15 bp, Artificial sequence
  Synthetic nucleotides for probe
tgattgcgttaaggg

SEQ ID NO: 616 - DNA, 15 bp, Artificial sequence
  Synthetic nucleotides for probe
acgcggcaaaggtta

SEQ ID NO: 617 - DNA, 15 bp, Artificial sequence
  Synthetic nucleotides for probe
tacgggttggagcta

SEQ ID NO: 618 - DNA, 15 bp, Artificial sequence
  Synthetic nucleotides for probe
tttcaacccgttcgg

SEQ ID NO: 619 - DNA, 15 bp, Artificial sequence
  Synthetic nucleotides for probe
tcgccgtgggattat

SEQ ID NO: 620 - DNA, 15 bp, Artificial sequence
  Synthetic nucleotides for probe
tagccctatgtggcg

SEQ ID NO: 621 - DNA, 15 bp, Artificial sequence
  Synthetic nucleotides for probe
atagttgtcccgccg

SEQ ID NO: 622 - DNA, 15 bp, Artificial sequence
  Synthetic nucleotides for probe
atttacgttcccgag

SEQ ID NO: 623 - DNA, 15 bp, Artificial sequence
  Synthetic nucleotides for probe
ttaaatcggctgacg

SEQ ID NO: 624 - DNA, 15 bp, Artificial sequence
  Synthetic nucleotides for probe
ttgtatcgtttgcga

SEQ ID NO: 625 - DNA, 15 bp, Artificial sequence
  Synthetic nucleotides for probe
tatctacaaatcgcg

SEQ ID NO: 626 - DNA, 15 bp, Artificial sequence
  Synthetic nucleotides for probe
tgcattgggccgtac

SEQ ID NO: 627 - DNA, 15 bp, Artificial sequence
  Synthetic nucleotides for probe
tacgtacccaatcgc

SEQ ID NO: 628 - DNA, 15 bp, Artificial sequence
  Synthetic nucleotides for probe
aaacgtcacgtccaa

SEQ ID NO: 629 - DNA, 15 bp, Artificial sequence
  Synthetic nucleotides for probe
taggcggcaatttcg

SEQ ID NO: 630 - DNA, 15 bp, Artificial sequence
  Synthetic nucleotides for probe
accttcgtttatcgt

SEQ ID NO: 631 - DNA, 15 bp, Artificial sequence
  Synthetic nucleotides for probe
tacgtttaccgtagc

SEQ ID NO: 632 - DNA, 15 bp, Artificial sequence
  Synthetic nucleotides for probe
attacctctttcgcg

SEQ ID NO: 633 - DNA, 15 bp, Artificial sequence
  Synthetic nucleotides for probe
tcgttttgcggtaat

SEQ ID NO: 634 - DNA, 15 bp, Artificial sequence
  Synthetic nucleotides for probe
tttcgactggggtat

SEQ ID NO: 635 - DNA, 15 bp, Artificial sequence
  Synthetic nucleotides for probe
acaaacggggttcga

SEQ ID NO: 636 - DNA, 15 bp, Artificial sequence
  Synthetic nucleotides for probe
tgcgctacgcgtttt

SEQ ID NO: 637 - DNA, 15 bp, Artificial sequence
  Synthetic nucleotides for probe
tatcggttaaaaccg

SEQ ID NO: 638 - DNA, 15 bp, Artificial sequence
  Synthetic nucleotides for probe
ttttcggtatgagcg

SEQ ID NO: 639 - DNA, 15 bp, Artificial sequence
  Synthetic nucleotides for probe
tcgcccgattttgtc

SEQ ID NO: 640 - DNA, 15 bp, Artificial sequence
  Synthetic nucleotides for probe
tcacggggcgtaaac

SEQ ID NO: 641 - DNA, 15 bp, Artificial sequence
  Synthetic nucleotides for probe
ataacccggggtcta

SEQ ID NO: 642 - DNA, 15 bp, Artificial sequence
  Synthetic nucleotides for probe
agcggggtaacgtat

SEQ ID NO: 643 - DNA, 15 bp, Artificial sequence
  Synthetic nucleotides for probe
aaaatcggatcagcg

SEQ ID NO: 644 - DNA, 15 bp, Artificial sequence
  Synthetic nucleotides for probe
tgatacgtccccgta

SEQ ID NO: 645 - DNA, 15 bp, Artificial sequence
  Synthetic nucleotides for probe
aggcgaaaattgcgt

SEQ ID NO: 646 - DNA, 15 bp, Artificial sequence
  Synthetic nucleotides for probe
tatcaccccgctacg

SEQ ID NO: 647 - DNA, 15 bp, Artificial sequence
  Synthetic nucleotides for probe
tggcgttttcgcgat

SEQ ID NO: 648 - DNA, 15 bp, Artificial sequence
  Synthetic nucleotides for probe
atcgtcgaaaattcg

SEQ ID NO: 649 - DNA, 15 bp, Artificial sequence
  Synthetic nucleotides for probe
tacgttccccgtatt

SEQ ID NO: 650 - DNA, 15 bp, Artificial sequence
  Synthetic nucleotides for probe
tattagctcgccccg

SEQ ID NO: 651 - DNA, 15 bp, Artificial sequence
  Synthetic nucleotides for probe
tagatcgacaaaacg

SEQ ID NO: 652 - DNA, 15 bp, Artificial sequence
  Synthetic nucleotides for probe
acctaacgcaacccc

SEQ ID NO: 653 - DNA, 15 bp, Artificial sequence
  Synthetic nucleotides for probe
ttttatcgccgcatg

SEQ ID NO: 654 - DNA, 15 bp, Artificial sequence
  Synthetic nucleotides for probe
aattaggggcgctta

SEQ ID NO: 655 - DNA, 15 bp, Artificial sequence
  Synthetic nucleotides for probe
acccctttacgcgtt

SEQ ID NO: 656 - DNA, 15 bp, Artificial sequence
  Synthetic nucleotides for probe
aaccccgtataattc

SEQ ID NO: 657 - DNA, 15 bp, Artificial sequence
  Synthetic nucleotides for probe
tagccgaaaagacgt

SEQ ID NO: 658 - DNA, 15 bp, Artificial sequence
  Synthetic nucleotides for probe
ttcgacgttttcgca

SEQ ID NO: 659 - DNA, 15 bp, Artificial sequence
  Synthetic nucleotides for probe
tatgtcggcaaaacg

SEQ ID NO: 660 - DNA, 15 bp, Artificial sequence
  Synthetic nucleotides for probe
tgtcggggtataacg

SEQ ID NO: 661 - DNA, 15 bp, Artificial sequence
  Synthetic nucleotides for probe
agcggggtatgagtt

SEQ ID NO: 662 - DNA, 15 bp, Artificial sequence
  Synthetic nucleotides for probe
ttttaagttcgtcgg

SEQ ID NO: 663 - DNA, 15 bp, Artificial sequence
  Synthetic nucleotides for probe
aggggccgtttatcg

SEQ ID NO: 664 - DNA, 15 bp, Artificial sequence
  Synthetic nucleotides for probe
taattttcacgcgtg

SEQ ID NO: 665 - DNA, 15 bp, Artificial sequence
  Synthetic nucleotides for probe
attgcgcggcaaaac

SEQ ID NO: 666 - DNA, 15 bp, Artificial sequence
  Synthetic nucleotides for probe
tcgactagccgtttt

SEQ ID NO: 667 - DNA, 15 bp, Artificial sequence
  Synthetic nucleotides for probe
acgggtaccccttgt

SEQ ID NO: 668 - DNA, 15 bp, Artificial sequence
  Synthetic nucleotides for probe
atttcgccccgatag

SEQ ID NO: 669 - DNA, 15 bp, Artificial sequence
  Synthetic nucleotides for probe
tgtaaaacgggtcgg

SEQ ID NO: 670 - DNA, 15 bp, Artificial sequence
  Synthetic nucleotides for probe
atatcgatagtgggg

SEQ ID NO: 671 - DNA, 15 bp, Artificial sequence
  Synthetic nucleotides for probe
agaacttttgtcgcg

SEQ ID NO: 672 - DNA, 15 bp, Artificial sequence
  Synthetic nucleotides for probe
tatttacccccggtc

SEQ ID NO: 673 - DNA, 15 bp, Artificial sequence
  Synthetic nucleotides for probe
ttacgtagggggatc

SEQ ID NO: 674 - DNA, 136 bp, Artificial sequence
  Synthetic nucleotides for capture probe
cggcaaactacgcgagccatacacgatactgcgcatagtgctctactcgcgaactcctgatctccatcctggctcaagtcaacagacgcgtgacgtaatatccggagctaattcctatagtgagtcgtattagctt

SEQ ID NO: 675 - DNA, 136 bp, Artificial sequence
  Synthetic nucleotides for capture probe
cggcaaactacgcgagccatacacgatactgcgcatagtgctctactcgcgaacgcttggaggtggctttccaggacaccaacagacgcgtgacgtaatatccggagctaattcctatagtgagtcgtattagctt

SEQ ID NO: 676 - DNA, 136 bp, Artificial sequence
  Synthetic nucleotides for capture probe
cggcaaactacgcgagccatacacgatactgcgcatagtgctctactcgcgaaccctcacagcacacggtgcagtaggactacagacgcgtgacgtaatatccggagctaattcctatagtgagtcgtattagctt

SEQ ID NO: 677 - DNA, 136 bp, Artificial sequence
  Synthetic nucleotides for capture probe
cggcaaactacgcgagccatacacgatactgcgcatagtgctctactcgcgaaacctccagacactccacacagaagcatcacagacgcgtgacgtaatatccggagctaattcctatagtgagtcgtattagctt

SEQ ID NO: 678 - DNA, 136 bp, Artificial sequence
  Synthetic nucleotides for capture probe
cggcaaactacgcgagccatacacgatactgcgcatagtgctctactcgcgaaagggttcctgcagcttggcatcctcagcacagacgcgtgacgtaatatccggagctaattcctatagtgagtcgtattagctt

SEQ ID NO: 679 - DNA, 136 bp, Artificial sequence
  Synthetic nucleotides for capture probe
cggcaaactacgcgagccatacacgatactgcgcatagtgctctactcgcgaaggcagcgctgagggaggcacatatagcaacagacgcgtgacgtaatatccggagctaattcctatagtgagtcgtattagctt

SEQ ID NO: 680 - DNA, 136 bp, Artificial sequence
  Synthetic nucleotides for capture probe
cggcaaactacgcgagccatacacgatactgcgcatagtgctctactcgcgaaatacccaactccttgagcaccaagtaccacagacgcgtgacgtaatatccggagctaattcctatagtgagtcgtattagctt

SEQ ID NO: 681 - DNA, 136 bp, Artificial sequence
  Synthetic nucleotides for capture probe
cggcaaactacgcgagccatacacgatactgcgcatagtgctctactcgcgaagatctggccttcatgcttaacagttcccacagacgcgtgacgtaatatccggagctaattcctatagtgagtcgtattagctt

SEQ ID NO: 682 - DNA, 136 bp, Artificial sequence
  Synthetic nucleotides for capture probe
cggcaaactacgcgagccatacacgatactgcgcatagtgctctactcgcgaacgttagagagatcattgcatgggcttccacagacgcgtgacgtaatatccggagctaattcctatagtgagtcgtattagctt

SEQ ID NO: 683 - DNA, 136 bp, Artificial sequence
  Synthetic nucleotides for capture probe
cggcaaactacgcgagccatacacgatactgcgcatagtgctctactcgcgaaaagtaccgggccctgtgagcagcagacaacagacgcgtgacgtaatatccggagctaattcctatagtgagtcgtattagctt

SEQ ID NO: 684 - DNA, 136 bp, Artificial sequence
  Synthetic nucleotides for capture probe
cggcaaactacgcgagccatacacgatactgcgcatagtgctctactcgcgaagaagccatcacgggcctgttcattccggacagacgcgtgacgtaatatccggagctaattcctatagtgagtcgtattagctt

SEQ ID NO: 685 - DNA, 136 bp, Artificial sequence
  Synthetic nucleotides for capture probe
cggcaaactacgcgagccatacacgatactgcgcatagtgctctactcgcgaatttgccctgtctgatggagttcgacttgacagacgcgtgacgtaatatccggagctaattcctatagtgagtcgtattagctt

SEQ ID NO: 686 - DNA, 136 bp, Artificial sequence
  Synthetic nucleotides for capture probe
cggcaaactacgcgagccatacacgatactgcgcatagtgctctactcgcgaaacgtcgtccttgccattcatgactacagacagacgcgtgacgtaatatccggagctaattcctatagtgagtcgtattagctt

SEQ ID NO: 687 - DNA, 136 bp, Artificial sequence
  Synthetic nucleotides for capture probe
cggcaaactacgcgagccatacacgatactgcgcatagtgctctactcgcgaaacaggtgtctgatgaccggtacactccaacagacgcgtgacgtaatatccggagctaattcctatagtgagtcgtattagctt

SEQ ID NO: 688 - DNA, 136 bp, Artificial sequence
  Synthetic nucleotides for capture probe
cggcaaactacgcgagccatacacgatactgcgcatagtgctctactcgcgaaaagcagccaggtctgagctgtgcacacgacagacgcgtgacgtaatatccggagctaattcctatagtgagtcgtattagctt

SEQ ID NO: 689 - DNA, 136 bp, Artificial sequence
  Synthetic nucleotides for capture probe
cggcaaactacgcgagccatacacgatactgcgcatagtgctctactcgcgaaggagatcccgcgtctggaaaggtatataacagacgcgtgacgtaatatccggagctaattcctatagtgagtcgtattagctt

SEQ ID NO: 690 - DNA, 136 bp, Artificial sequence
  Synthetic nucleotides for capture probe
cggcaaactacgcgagccatacacgatactgcgcatagtgctctactcgcgaagcagcatgaacctgagtactaagagagcacagacgcgtgacgtaatatccggagctaattcctatagtgagtcgtattagctt

SEQ ID NO: 691 - DNA, 136 bp, Artificial sequence
  Synthetic nucleotides for capture probe
cggcaaactacgcgagccatacacgatactgcgcatagtgctctactcgcgaatccagcaaatgtggagcacgggttacttacagacgcgtgacgtaatatccggagctaattcctatagtgagtcgtattagctt

SEQ ID NO: 692 - DNA, 136 bp, Artificial sequence
  Synthetic nucleotides for capture probe
cggcaaactacgcgagccatacacgatactgcgcatagtgctctactcgcgaaccttgctcatctgagcccacattcacaaacagacgcgtgacgtaatatccggagctaattcctatagtgagtcgtattagctt

SEQ ID NO: 693 - DNA, 136 bp, Artificial sequence
  Synthetic nucleotides for capture probe
cggcaaactacgcgagccatacacgatactgcgcatagtgctctactcgcgaatgcagctttcttatctccagtgatgcccacagacgcgtgacgtaatatccggagctaattcctatagtgagtcgtattagctt

SEQ ID NO: 694 - DNA, 136 bp, Artificial sequence
  Synthetic nucleotides for capture probe
cggcaaactacgcgagccatacacgatactgcgcatagtgctctactcgcgaattgacctgcggcctctggtctctggtgtacagacgcgtgacgtaatatccggagctaattcctatagtgagtcgtattagctt

SEQ ID NO: 695 - DNA, 136 bp, Artificial sequence
  Synthetic nucleotides for capture probe
cggcaaactacgcgagccatacacgatactgcgcatagtgctctactcgcgaatccatctcctgtcatgtcctgcgtgtaaacagacgcgtgacgtaatatccggagctaattcctatagtgagtcgtattagctt

SEQ ID NO: 696 - DNA, 136 bp, Artificial sequence
  Synthetic nucleotides for capture probe
cggcaaactacgcgagccatacacgatactgcgcatagtgctctactcgcgaacttggtctcacgggtgagctttggcattacagacgcgtgacgtaatatccggagctaattcctatagtgagtcgtattagctt

SEQ ID NO: 697 - DNA, 136 bp, Artificial sequence
  Synthetic nucleotides for capture probe
cggcaaactacgcgagccatacacgatactgcgcatagtgctctactcgcgaagtagccggaaactccacagggtactcctacagacgcgtgacgtaatatccggagctaattcctatagtgagtcgtattagctt

SEQ ID NO: 698 - DNA, 136 bp, Artificial sequence
  Synthetic nucleotides for capture probe
cggcaaactacgcgagccatacacgatactgcgcatagtgctctactcgcgaatgtcacttcttccatgaagtcgacgctgacagacgcgtgacgtaatatccggagctaattcctatagtgagtcgtattagctt

SEQ ID NO: 699 - DNA, 136 bp, Artificial sequence
  Synthetic nucleotides for capture probe
cggcaaactacgcgagccataatcgtatatcgccttacgataatagaaccgaatgtgccagtctatgacattcccagacacagcgtatatagtggttacgccgttacatcagtcctatagtgagtcgtattagctt

SEQ ID NO: 700 - DNA, 136 bp, Artificial sequence
  Synthetic nucleotides for capture probe
cggcaaactacgcgagccataatcgtatatcgccttacgataatagaaccgaaccacagctcaggttgccctcggctttcaagcgtatatagtggttacgccgttacatcagtcctatagtgagtcgtattagctt

SEQ ID NO: 701 - DNA, 136 bp, Artificial sequence
  Synthetic nucleotides for capture probe
cggcaaactacgcgagccataatcgtatatcgccttacgataatagaaccgaacttgaacagttggaagtgtcaacagggcagcgtatatagtggttacgccgttacatcagtcctatagtgagtcgtattagctt

SEQ ID NO: 702 - DNA, 136 bp, Artificial sequence
  Synthetic nucleotides for capture probe
cggcaaactacgcgagccataatcgtatatcgccttacgataatagaaccgaattagagtggagccgagggtgatgtcaatagcgtatatagtggttacgccgttacatcagtcctatagtgagtcgtattagctt

SEQ ID NO: 703 - DNA, 136 bp, Artificial sequence
  Synthetic nucleotides for capture probe
cggcaaactacgcgagccataatcgtatatcgccttacgataatagaaccgaagatgagactccaagggccaaattctgtgagcgtatatagtggttacgccgttacatcagtcctatagtgagtcgtattagctt

SEQ ID NO: 704 - DNA, 136 bp, Artificial sequence
  Synthetic nucleotides for capture probe
cggcaaactacgcgagccataatcgtatatcgccttacgataatagaaccgaaggatctgtctgtccgttcccgaagtccaagcgtatatagtggttacgccgttacatcagtcctatagtgagtcgtattagctt

SEQ ID NO: 705 - DNA, 136 bp, Artificial sequence
  Synthetic nucleotides for capture probe
cggcaaactacgcgagccataatcgtatatcgccttacgataatagaaccgaatcaagctccaccgaagaagatcccggctagcgtatatagtggttacgccgttacatcagtcctatagtgagtcgtattagctt

SEQ ID NO: 706 - DNA, 136 bp, Artificial sequence
  Synthetic nucleotides for capture probe
cggcaaactacgcgagccataatcgtatatcgccttacgataatagaaccgaaaaggtaccggaaggattggacaggacaaagcgtatatagtggttacgccgttacatcagtcctatagtgagtcgtattagctt

SEQ ID NO: 707 - DNA, 136 bp, Artificial sequence
  Synthetic nucleotides for capture probe
cggcaaactacgcgagccataatcgtatatcgccttacgataatagaaccgaaggcactccttggaagatccatcagaactagcgtatatagtggttacgccgttacatcagtcctatagtgagtcgtattagctt

SEQ ID NO: 708 - DNA, 136 bp, Artificial sequence
  Synthetic nucleotides for capture probe
cggcaaactacgcgagccataatcgtatatcgccttacgataatagaaccgaatcccacagatctgcaccatgaccacaatagcgtatatagtggttacgccgttacatcagtcctatagtgagtcgtattagctt

SEQ ID NO: 709 - DNA, 136 bp, Artificial sequence
  Synthetic nucleotides for capture probe
cggcaaactacgcgagccataatcgtatatcgccttacgataatagaaccgaacgcctccactgtttctgaacattctcctagcgtatatagtggttacgccgttacatcagtcctatagtgagtcgtattagctt

SEQ ID NO: 710 - DNA, 136 bp, Artificial sequence
  Synthetic nucleotides for capture probe
cggcaaactacgcgagccataatcgtatatcgccttacgataatagaaccgaacccaggttatcggagctcttcttgatgaagcgtatatagtggttacgccgttacatcagtcctatagtgagtcgtattagctt

SEQ ID NO: 711 - DNA, 136 bp, Artificial sequence
  Synthetic nucleotides for capture probe
cggcaaactacgcgagccataatcgtatatcgccttacgataatagaaccgaaggacgggaatgattgacgtctgttctccagcgtatatagtggttacgccgttacatcagtcctatagtgagtcgtattagctt

SEQ ID NO: 712 - DNA, 136 bp, Artificial sequence
  Synthetic nucleotides for capture probe
cggcaaactacgcgagccataatcgtatatcgccttacgataatagaaccgaagacattccaccggcgtagctttccgtgcagcgtatatagtggttacgccgttacatcagtcctatagtgagtcgtattagctt

SEQ ID NO: 713 - DNA, 136 bp, Artificial sequence
  Synthetic nucleotides for capture probe
cggcaaactacgcgagccataatcgtatatcgccttacgataatagaaccgaatattcttgccgggctcagagtgttctcaagcgtatatagtggttacgccgttacatcagtcctatagtgagtcgtattagctt

SEQ ID NO: 714 - DNA, 136 bp, Artificial sequence
  Synthetic nucleotides for capture probe
cggcaaactacgcgagccataatcgtatatcgccttacgataatagaaccgaaaggccactgccaagcctaactatgaggtagcgtatatagtggttacgccgttacatcagtcctatagtgagtcgtattagctt

SEQ ID NO: 715 - DNA, 136 bp, Artificial sequence
  Synthetic nucleotides for capture probe
cggcaaactacgcgagccataatcgtatatcgccttacgataatagaaccgaaaatggagatgcttaggctgcgtgtcttgagcgtatatagtggttacgccgttacatcagtcctatagtgagtcgtattagctt

SEQ ID NO: 716 - DNA, 136 bp, Artificial sequence
  Synthetic nucleotides for capture probe
cggcaaactacgcgagccataatcgtatatcgccttacgataatagaaccgaagccacagtctgatccatgcatattccacagcgtatatagtggttacgccgttacatcagtcctatagtgagtcgtattagctt

SEQ ID NO: 717 - DNA, 136 bp, Artificial sequence
  Synthetic nucleotides for capture probe
cggcaaactacgcgagccataatcgtatatcgccttacgataatagaaccgaattgggctcaacctacaccctcactaacaagcgtatatagtggttacgccgttacatcagtcctatagtgagtcgtattagctt

SEQ ID NO: 718 - DNA, 136 bp, Artificial sequence
  Synthetic nucleotides for capture probe
cggcaaactacgcgagccataatcgtatatcgccttacgataatagaaccgaaagcatgcactgaggcccatgaataggacagcgtatatagtggttacgccgttacatcagtcctatagtgagtcgtattagctt

SEQ ID NO: 719 - DNA, 136 bp, Artificial sequence
  Synthetic nucleotides for capture probe
cggcaaactacgcgagccataatcgtatatcgccttacgataatagaaccgaaaaagttcaggtctgccaagatggcagtcagcgtatatagtggttacgccgttacatcagtcctatagtgagtcgtattagctt

SEQ ID NO: 720 - DNA, 136 bp, Artificial sequence
  Synthetic nucleotides for capture probe
cggcaaactacgcgagccataatcgtatatcgccttacgataatagaaccgaaaggacacagcaactctgatgtagctggcagcgtatatagtggttacgccgttacatcagtcctatagtgagtcgtattagctt

SEQ ID NO: 721 - DNA, 136 bp, Artificial sequence
  Synthetic nucleotides for capture probe
cggcaaactacgcgagccataatcgtatatcgccttacgataatagaaccgaagctctgctgaggtgaatcttagtcacctagcgtatatagtggttacgccgttacatcagtcctatagtgagtcgtattagctt

SEQ ID NO: 722 - DNA, 136 bp, Artificial sequence
  Synthetic nucleotides for capture probe
cggcaaactacgcgagccataatcgtatatcgccttacgataatagaaccgaacagctgtgtgtagcctgaactctgggtcagcgtatatagtggttacgccgttacatcagtcctatagtgagtcgtattagctt

SEQ ID NO: 723 - DNA, 136 bp, Artificial sequence
  Synthetic nucleotides for capture probe
cggcaaactacgcgagccataatcgtatatcgccttacgataatagaaccgaacacatcacagtgaaaggagagggtgggaagcgtatatagtggttacgccgttacatcagtcctatagtgagtcgtattagctt

SEQ ID NO: 724 - DNA, 136 bp, Artificial sequence
  Synthetic nucleotides for capture probe
cggcaaactacgcgagccataatcgtatatcgccttacgataatagaaccgaataggagaaagctgtccagtcaccaccttagcgtatatagtggttacgccgttacatcagtcctatagtgagtcgtattagctt

SEQ ID NO: 725 - DNA, 136 bp, Artificial sequence
  Synthetic nucleotides for capture probe
cggcaaactacgcgagccataatcgtatatcgccttacgataatagaaccgaaacaagcatcttgagccagagatggacagagcgtatatagtggttacgccgttacatcagtcctatagtgagtcgtattagctt

SEQ ID NO: 726 - DNA, 136 bp, Artificial sequence
  Synthetic nucleotides for capture probe
cggcaaactacgcgagccataatcgtatatcgccttacgataatagaaccgaatgtcctctttgtccttcacaggtaacgcagcgtatatagtggttacgccgttacatcagtcctatagtgagtcgtattagctt

SEQ ID NO: 727 - DNA, 136 bp, Artificial sequence
  Synthetic nucleotides for capture probe
cggcaaactacgcgagccataatcgtatatcgccttacgataatagaaccgaaccacacaagacagagctgctccaagtttagcgtatatagtggttacgccgttacatcagtcctatagtgagtcgtattagctt

SEQ ID NO: 728 - DNA, 136 bp, Artificial sequence
  Synthetic nucleotides for capture probe
cggcaaactacgcgagccatacgcctattcgccaataagacgaactagcgaaatgcctctacctgagctaatccttgctgaatcgctagtggtaagtacgactattgagaccacctatagtgagtcgtattagctt

SEQ ID NO: 729 - DNA, 136 bp, Artificial sequence
  Synthetic nucleotides for capture probe
cggcaaactacgcgagccatacgcctattcgccaataagacgaactagcgaaacgccctgcaacagatactggagcagcagatcgctagtggtaagtacgactattgagaccacctatagtgagtcgtattagctt

SEQ ID NO: 730 - DNA, 136 bp, Artificial sequence
  Synthetic nucleotides for capture probe
cggcaaactacgcgagccatacgcctattcgccaataagacgaactagcgaaatcgttctcccgctcttgctgcgtctcctatcgctagtggtaagtacgactattgagaccacctatagtgagtcgtattagctt

SEQ ID NO: 731 - DNA, 136 bp, Artificial sequence
  Synthetic nucleotides for capture probe
cggcaaactacgcgagccatacgcctattcgccaataagacgaactagcgaaatcatgaccaacgggctgccagagacagcatcgctagtggtaagtacgactattgagaccacctatagtgagtcgtattagctt

SEQ ID NO: 732 - DNA, 136 bp, Artificial sequence
  Synthetic nucleotides for capture probe
cggcaaactacgcgagccatacgcctattcgccaataagacgaactagcgaaattcgttccagtccggcaactcatcccggatcgctagtggtaagtacgactattgagaccacctatagtgagtcgtattagctt

SEQ ID NO: 733 - DNA, 136 bp, Artificial sequence
  Synthetic nucleotides for capture probe
cggcaaactacgcgagccatacgcctattcgccaataagacgaactagcgaaaaaacacctcatcctcctcccgatcccagatcgctagtggtaagtacgactattgagaccacctatagtgagtcgtattagctt

SEQ ID NO: 734 - DNA, 136 bp, Artificial sequence
  Synthetic nucleotides for capture probe
cggcaaactacgcgagccatacgcctattcgccaataagacgaactagcgaaagtgtccgcggccgaatgtagtttgggaaatcgctagtggtaagtacgactattgagaccacctatagtgagtcgtattagctt

SEQ ID NO: 735 - DNA, 136 bp, Artificial sequence
  Synthetic nucleotides for capture probe
cggcaaactacgcgagccatacgcctattcgccaataagacgaactagcgaaacgcaggtggcaacgcgtgatggaagtgaatcgctagtggtaagtacgactattgagaccacctatagtgagtcgtattagctt

SEQ ID NO: 736 - DNA, 136 bp, Artificial sequence
  Synthetic nucleotides for capture probe
cggcaaactacgcgagccatacgcctattcgccaataagacgaactagcgaaaagaagaggacggatgccggcaacgtgaaatcgctagtggtaagtacgactattgagaccacctatagtgagtcgtattagctt

SEQ ID NO: 737 - DNA, 136 bp, Artificial sequence
  Synthetic nucleotides for capture probe
cggcaaactacgcgagccatacgcctattcgccaataagacgaactagcgaaaagtctgacaggtccggtgccgacagaacatcgctagtggtaagtacgactattgagaccacctatagtgagtcgtattagctt

SEQ ID NO: 738 - DNA, 136 bp, Artificial sequence
  Synthetic nucleotides for capture probe
cggcaaactacgcgagccatacgcctattcgccaataagacgaactagcgaaagtcctagaagctgggctcagctgggtcaatcgctagtggtaagtacgactattgagaccacctatagtgagtcgtattagctt

SEQ ID NO: 739 - DNA, 136 bp, Artificial sequence
  Synthetic nucleotides for capture probe
cggcaaactacgcgagccatacgcctattcgccaataagacgaactagcgaaatttcccgtctgggactgggaagtcgctaatcgctagtggtaagtacgactattgagaccacctatagtgagtcgtattagctt

SEQ ID NO: 740 - DNA, 136 bp, Artificial sequence
  Synthetic nucleotides for capture probe
cggcaaactacgcgagccatacgcctattcgccaataagacgaactagcgaaagagaaggagaagtgggtaagttcacagcatcgctagtggtaagtacgactattgagaccacctatagtgagtcgtattagctt

SEQ ID NO: 741 - DNA, 136 bp, Artificial sequence
  Synthetic nucleotides for capture probe
cggcaaactacgcgagccatacgcctattcgccaataagacgaactagcgaaatttggccgggacactgcgtcctcagctaatcgctagtggtaagtacgactattgagaccacctatagtgagtcgtattagctt

SEQ ID NO: 742 - DNA, 136 bp, Artificial sequence
  Synthetic nucleotides for capture probe
cggcaaactacgcgagccatacgcctattcgccaataagacgaactagcgaaaattccgagcagctcggacctctggtacgatcgctagtggtaagtacgactattgagaccacctatagtgagtcgtattagctt

SEQ ID NO: 743 - DNA, 136 bp, Artificial sequence
  Synthetic nucleotides for capture probe
cggcaaactacgcgagccatacgcctattcgccaataagacgaactagcgaaatggaagagctctccctggtcctgaggctatcgctagtggtaagtacgactattgagaccacctatagtgagtcgtattagctt

SEQ ID NO: 744 - DNA, 136 bp, Artificial sequence
  Synthetic nucleotides for capture probe
cggcaaactacgcgagccatacgcctattcgccaataagacgaactagcgaaagacggtccagtgcctgcaacagtaccgaatcgctagtggtaagtacgactattgagaccacctatagtgagtcgtattagctt

SEQ ID NO: 745 - DNA, 136 bp, Artificial sequence
  Synthetic nucleotides for capture probe
cggcaaactacgcgagccatacgcctattcgccaataagacgaactagcgaaagagcttctgctgcttcttcgggtgttccatcgctagtggtaagtacgactattgagaccacctatagtgagtcgtattagctt

SEQ ID NO: 746 - DNA, 136 bp, Artificial sequence
  Synthetic nucleotides for capture probe
cggcaaactacgcgagccatacgcctattcgccaataagacgaactagcgaaactggagtatgagcgatggtcgagggctgatcgctagtggtaagtacgactattgagaccacctatagtgagtcgtattagctt

SEQ ID NO: 747 - DNA, 136 bp, Artificial sequence
  Synthetic nucleotides for capture probe
cggcaaactacgcgagccatacgcctattcgccaataagacgaactagcgaaagcttggatttctggtgccgggaggctatatcgctagtggtaagtacgactattgagaccacctatagtgagtcgtattagctt

SEQ ID NO: 748 - DNA, 136 bp, Artificial sequence
  Synthetic nucleotides for capture probe
cggcaaactacgcgagccatacgcctattcgccaataagacgaactagcgaaaaaggatgctagcgcctccagctcttctgatcgctagtggtaagtacgactattgagaccacctatagtgagtcgtattagctt

SEQ ID NO: 749 - DNA, 136 bp, Artificial sequence
  Synthetic nucleotides for capture probe
cggcaaactacgcgagccatacgcctattcgccaataagacgaactagcgaaactcttgttggcgcttagcattgctcggaatcgctagtggtaagtacgactattgagaccacctatagtgagtcgtattagctt

SEQ ID NO: 750 - DNA, 136 bp, Artificial sequence
  Synthetic nucleotides for capture probe
cggcaaactacgcgagccatacgcctattcgccaataagacgaactagcgaaatcagcgtgtgcgtgcgggtttcagtctcatcgctagtggtaagtacgactattgagaccacctatagtgagtcgtattagctt

SEQ ID NO: 751 - DNA, 136 bp, Artificial sequence
  Synthetic nucleotides for capture probe
cggcaaactacgcgagccatacgcctattcgccaataagacgaactagcgaaagctttcggacattcgagcctggaattggatcgctagtggtaagtacgactattgagaccacctatagtgagtcgtattagctt